European Patent Specification EP 3 514 226 B1, published March 29, 2023. Title: COMPOSITIONS AND METHODS FOR THE BIOSYNTHESIS OF VANILLIN OR VANILLIN BETA-D-GLUCOSIDE. Applicant: Hansen, Joergen Hansen, Esben H. Sompalli, Honey Polur Sheridan, Joseph M. Heal, Jonathan R. Hamilton, William D.O. The sequence listing filed with the application follows.

SEQUENCE LISTING (56 sequences)

SEQ ID NO: 1 - DNA, 3912 bp, Saccharomyces cerevisiae
atggtgcagttagccaaagtcccaattctaggaaatgatattatccacgttgggtataacattcatgaccatttggttgaaaccataattaaacattgtccttcttcgacatacgttatttgcaatgatacgaacttgagtaaagttccatactaccagcaattagtcctggaattcaaggcttctttgccagaaggctctcgtttacttacttatgttgttaaaccaggtgagacaagtaaaagtagagaaaccaaagcgcagctagaagattatcttttagtggaaggatgtactcgtgatacggttatggtagcgatcggtggtggtgttattggtgacatgattgggttcgttgcatctacatttatgagaggtgttcgtgttgtccaagtaccaacatccttattggcaatggtcgattcctccattggtggtaaaactgctattgacactcctctaggtaaaaactttattggtgcattttggcaaccaaaatttgtccttgtagatattaaatggctagaaacgttagccaagagagagtttatcaatgggatggcagaagttatcaagactgcttgtatttggaacgctgacgaatttactagattagaatcaaacgcttcgttgttcttaaatgttgttaatggggcaaaaaatgtcaaggttaccaatcaattgacaaacgagattgacgagatatcgaatacagatattgaagctatgttggatcatacatataagttagttcttgagagtattaaggtcaaagcggaagttgtctcttcggatgaacgtgaatccagtctaagaaaccttttgaacttcggacattctattggtcatgcttatgaagctatactaaccccacaagcattacatggtgaatgtgtgtccattggtatggttaaagaggcggaattatcccgttatttcggtattctctcccctacccaagttgcacgtctatccaagattttggttgcctacgggttgcctgtttcgcctgatgagaaatggtttaaagagctaaccttacataagaaaacaccattggatatcttattgaagaaaatgagtattgacaagaaaaacgagggttccaaaaagaaggtggtcattttagaaagtattggtaagtgctatggtgactccgctcaatttgttagcgatgaagacctgagatttattctaacagatgaaaccctcgtttaccccttcaaggacatccctgctgatcaacagaaagttgttatcccccctggttctaagtccatctccaatcgtgctttaattcttgctgccctcggtgaaggtcaatgtaaaatcaagaacttattacattctgatgatactaaacatatgttaaccgctgttcatgaattgaaaggtgctacgatatcatgggaagataatggtgagacggtagtggtggaaggacatggtggttccacattgtcagcttgtgctgaccccttatatctaggtaatgcaggtactgcatctagatttttgacttccttggctgccttggtcaattctacttcaagccaaaagtatatcgttttaactggtaacgcaagaatgcaacaaagaccaattgctcctttggtcgattctttgcgtgctaatggtactaaaattgagtacttgaataatgaaggttccctgccaatcaaagtttatactgattcggtattcaaaggtggtagaattgaattagctgctacagtttcttctcagtacgtatcctctatcttgatgtgtgccccatacgctgaagaacctgtaactttggctcttgttggtggtaagccaatctctaaattgtacgtcgatatgacaataaaaatgatggaaaaattcggtatcaatgttgaaacttctactacagaaccttacacttattatattccaaagggacattatattaacccatcagaatacgtcattgaaagtgatgcctcaagtgctacatacccattggccttcgccgcaatgactggtactaccgtaacggttccaaacattggttttgagtcgttacaaggtgatgccagatttgcaagagatgtcttgaaacctatgggttgtaaaataactcaaacggcaacttcaactactgtttcgggtcctcctgtaggtactttaaagccattaaaacatgttgatatggagccaatgactgatgcgttcttaactgcatgtgttgttgccgctatttcgcacgacagtgatccaaattctgcaaatacaaccaccattgaaggtattgcaaaccagcgtgtcaaagagtgtaacagaattttggccatggctacagagctcgccaaatttggcgtcaaaactacagaattaccagatggtattcaagtccatggtttaaactcgataaaagatttgaaggttccttccgactcttctggacctgtcggtgtatgcacatatgatgatcatcgtgtggccatgagtttctcgcttcttgcaggaatggtaaattctcaaaatgaacgtgacgaagttgctaatcctgtaagaatacttgaaagacattgtactggtaaaacctggcctggctggtgggatgtgttacattccgaactaggtgccaaattagatggtgcagaacctttagagtgcacatccaaaaagaactcaaagaaaagcgttgtcattattggcatgagagcagctggcaaaactactataagtaaatggtgcgcatccgctctgggttacaaattagttgacctagacgagctgtttgagcaacagcataacaatcaaagtgttaaacaatttgttgtggagaacggttgggagaagttccgtgaggaagaaacaagaattttcaaggaagttattcaaaattacggcgatgatggatatgttttctcaacaggtggcggtattgttgaaagcgctgagtctagaaaagccttaaaagattttgcctcatcaggtggatacgttttacacttacatagggatattgaggagacaattgtctttttacaaagtgatccttcaagacctgcctatgtggaagaaattcgtgaagtttggaacagaagggaggggtggtataaagaatgctcaaatttctctttctttgctcctcattgctccgcagaagctgagttccaagctctaagaagatcgtttagtaagtacattgcaaccattacaggtgtcagagaaatagaaattccaagcggaagatctgcctttgtgtgtttaacctttgatgacttaactgaacaaactgagaatttgactccaatctgttatggttgtgaggctgtagaggtcagagtagaccatttggctaattactctgctgatttcgtgagtaaacagttatctatattgcgtaaagccactgacagtattcctatcatttttactgtgcgaaccatgaagcaaggtggcaactttcctgatgaagagttcaaaaccttgagagagctatacgatattgccttgaagaatggtgttgaattccttgacttagaactaactttacctactgatatccaatatgaggttattaacaaaaggggcaacaccaagatcattggttcccatcatgacttccaaggattatactcctgggacgacgctgaatgggaaaacagattcaatcaagcgttaactcttgatgtggatgttgtaaaatttgtgggtacggctgttaatttcgaagataatttgagactggaacactttagggatacacacaagaataagcctttaattgcagttaatatgacttctaaaggtagcatttctcgtgttttgaataatgttttaacacctgtgacatcagatttattgcctaactccgctgcccctggccaattgacagtagcacaaattaacaagatgtatacatctatgggaggttga

SEQ ID NO: 2 - protein, 1303 aa, Saccharomyces cerevisiae
MVQLAKVPILGNDIIHVGYNIHDHLVETIIKHCPSSTYVICNDTNLSKVPYYQQLVLEFKASLPEGSRLLTYVVKPGETSKSRETKAQLEDYLLVEGCTRDTVMVAIGGGVIGDMIGFVASTFMRGVRVVQVPTSLLAMVDSSIGGKTAIDTPLGKNFIGAFWQPKFVLVDIKWLETLAKREFINGMAEVIKTACIWNADEFTRLESNASLFLNVVNGAKNVKVTNQLTNEIDEISNTDIEAMLDHTYKLVLESIKVKAEVVSSDERESSLRNLLNFGHSIGHAYEAILTPQALHGECVSIGMVKEAELSRYFGILSPTQVARLSKILVAYGLPVSPDEKWFKELTLHKKTPLDILLKKMSIDKKNEGSKKKVVILESIGKCYGDSAQFVSDEDLRFILTDETLVYPFKDIPADQQKVVIPPGSKSISNRALILAALGEGQCKIKNLLHSDDTKHMLTAVHELKGATISWEDNGETVVVEGHGGSTLSACADPLYLGNAGTASRFLTSLAALVNSTSSQKYIVLTGNARMQQRPIAPLVDSLRANGTKIEYLNNEGSLPIKVYTDSVFKGGRIELAATVSSQYVSSILMCAPYAEEPVTLALVGGKPISKLYVDMTIKMMEKFGINVETSTTEPYTYYIPKGHYINPSEYVIESDASSATYPLAFAAMTGTTVTVPNIGFESLQGDARFARDVLKPMGCKITQTATSTTVSGPPVGTLKPLKHVDMEPMTDAFLTACVVAAISHDSDPNSANTTTIEGIANQRVKECNRILAMATELAKFGVKTTELPDGIQVHGLNSIKDLKVPSDSSGPVGVCTYDDHRVAMSFSLLAGMVNSQNERDEVANPVRILERHCTGKTWPGWWDVLHSELGAKLDGAEPLECTSKKNSKKSVVIIGMRAAGKTTISKWCASALGYKLVDLDELFEQQHNNQSVKQFVVENGWEKFREEETRIFKEVIQNYGDDGYVFSTGGGIVESAESRKALKDFASSGGYVLHLHRDIEETIVFLQSDPSRPAYVEEIREVWNRREGWYKECSNFSFFAPHCSAEAEFQALRRSFSKYIATITGVREIEIPSGRSAFVCLTFDDLTEQTENLTPICYGCEAVEVRVDHLANYSADFVSKQLSILRKATDSIPIIFTVRTMKQGGNFPDEEFKTLRELYDIALKNGVEFLDLELTLPTDIQYEVINKRGNTKIIGSHHDFQGLYSWDDAEWENRFNQALTLDVDVVKFVGTAVNFEDNLRLEHFRDTHKNKPLIAVNMTSKGSISRVLNNVLTPVTSDLLPNSAAPGQLTVAQINKMYTSMGG

SEQ ID NO: 3 - DNA, 4767 bp, Saccharomyces cerevisiae
atggtgcagttagccaaagtcccaattctaggaaatgatattatccacgttgggtataacattcatgaccatttggttgaaaccataattaaacattgtccttcttcgacatacgttatttgcaatgatacgaacttgagtaaagttccatactaccagcaattagtcctggaattcaaggcttctttgccagaaggctctcgtttacttacttatgttgttaaaccaggtgagacaagtaaaagtagagaaaccaaagcgcagctagaagattatcttttagtggaaggatgtactcgtgatacggttatggtagcgatcggtggtggtgttattggtgacatgattgggttcgttgcatctacatttatgagaggtgttcgtgttgtccaagtaccaacatccttattggcaatggtcgattcctccattggtggtaaaactgctattgacactcctctaggtaaaaactttattggtgcattttggcaaccaaaatttgtccttgtagatattaaatggctagaaacgttagccaagagagagtttatcaatgggatggcagaagttatcaagactgcttgtatttggaacgctgacgaatttactagattagaatcaaacgcttcgttgttcttaaatgttgttaatggggcaaaaaatgtcaaggttaccaatcaattgacaaacgagattgacgagatatcgaatacagatattgaagctatgttggatcatacatataagttagttcttgagagtattaaggtcaaagcggaagttgtctcttcggatgaacgtgaatccagtctaagaaaccttttgaacttcggacattctattggtcatgcttatgaagctatactaaccccacaagcattacatggtgaatgtgtgtccattggtatggttaaagaggcggaattatcccgttatttcggtattctctcccctacccaagttgcacgtctatccaagattttggttgcctacgggttgcctgtttcgcctgatgagaaatggtttaaagagctaaccttacataagaaaacaccattggatatcttattgaagaaaatgagtattgacaagaaaaacgagggttccaaaaagaaggtggtcattttagaaagtattggtaagtgctatggtgactccgctcaatttgttagcgatgaagacctgagatttattctaacagatgaaaccctcgtttaccccttcaaggacatccctgctgatcaacagaaagttgttatcccccctggttctaagtccatctccaatcgtgctttaattcttgctgccctcggtgaaggtcaatgtaaaatcaagaacttattacattctgatgatactaaacatatgttaaccgctgttcatgaattgaaaggtgctacgatatcatgggaagataatggtgagacggtagtggtggaaggacatggtggttccacattgtcagcttgtgctgaccccttatatctaggtaatgcaggtactgcatctagatttttgacttccttggctgccttggtcaattctacttcaagccaaaagtatatcgttttaactggtaacgcaagaatgcaacaaagaccaattgctcctttggtcgattctttgcgtgctaatggtactaaaattgagtacttgaataatgaaggttccctgccaatcaaagtttatactgattcggtattcaaaggtggtagaattgaattagctgctacagtttcttctcagtacgtatcctctatcttgatgtgtgccccatacgctgaagaacctgtaactttggctcttgttggtggtaagccaatctctaaattgtacgtcgatatgacaataaaaatgatggaaaaattcggtatcaatgttgaaacttctactacagaaccttacacttattatattccaaagggacattatattaacccatcagaatacgtcattgaaagtgatgcctcaagtgctacatacccattggccttcgccgcaatgactggtactaccgtaacggttccaaacattggttttgagtcgttacaaggtgatgccagatttgcaagagatgtcttgaaacctatgggttgtaaaataactcaaacggcaacttcaactactgtttcgggtcctcctgtaggtactttaaagccattaaaacatgttgatatggagccaatgactgatgcgttcttaactgcatgtgttgttgccgctatttcgcacgacagtgatccaaattctgcaaatacaaccaccattgaaggtattgcaaaccagcgtgtcaaagagtgtaacagaattttggccatggctacagagctcgccaaatttggcgtcaaaactacagaattaccagatggtattcaagtccatggtttaaactcgataaaagatttgaaggttccttccgactcttctggacctgtcggtgtatgcacatatgatgatcatcgtgtggccatgagtttctcgcttcttgcaggaatggtaaattctcaaaatgaacgtgacgaagttgctaatcctgtaagaatacttgaaagacattgtactggtaaaacctggcctggctggtgggatgtgttacattccgaactaggtgccaaattagatggtgcagaacctttagagtgcacatccaaaaagaactcaaagaaaagcgttgtcattattggcatgagagcagctggcaaaactactataagtaaatggtgcgcatccgctctgggttacaaattagttgacctagacgagctgtttgagcaacagcataacaatcaaagtgttaaacaatttgttgtggagaacggttgggagaagttccgtgaggaagaaacaagaattttcaaggaagttattcaaaattacggcgatgatggatatgttttctcaacaggtggcggtattgttgaaagcgctgagtctagaaaagccttaaaagattttgcctcatcaggtggatacgttttacacttacatagggatattgaggagacaattgtctttttacaaagtgatccttcaagacctgcctatgtggaagaaattcgtgaagtttggaacagaagggaggggtggtataaagaatgctcaaatttctctttctttgctcctcattgctccgcagaagctgagttccaagctctaagaagatcgtttagtaagtacattgcaaccattacaggtgtcagagaaatagaaattccaagcggaagatctgcctttgtgtgtttaacctttgatgacttaactgaacaaactgagaatttgactccaatctgttatggttgtgaggctgtagaggtcagagtagaccatttggctaattactctgctgatttcgtgagtaaacagttatctatattgcgtaaagccactgacagtattcctatcatttttactgtgcgaaccatgaagcaaggtggcaactttcctgatgaagagttcaaaaccttgagagagctatacgatattgccttgaagaatggtgttgaattccttgacttagaactaactttacctactgatatccaatatgaggttattaacaaaaggggcaacaccaagatcattggttcccatcatgacttccaaggattatactcctgggacgacgctgaatgggaaaacagattcaatcaagcgttaactcttgatgtggatgttgtaaaatttgtgggtacggctgttaatttcgaagataatttgagactggaacactttagggatacacacaagaataagcctttaattgcagttaatatgacttctaaaggtagcatttctcgtgttttgaataatgttttaacacctgtgacatcagatttattgcctaactccgctgcccctggccaattgacagtagcacaaattaacaagatgtatacatctatgggaggtatcgagcctaaggaactgtttgttgttggaaagccaattggccactctagatcgccaattttacataacactggctatgaaattttaggtttacctcacaagttcgataaatttgaaactgaatccgcacaattggtgaaagaaaaacttttggacggaaacaagaactttggcggtgctgcagtcacaattcctctgaaattagatataatgcagtacatggatgaattgactgatgctgctaaagttattggtgctgtaaacacagttataccattgggtaacaagaagtttaagggtgataataccgactggttaggtatccgtaatgccttaattaacaatggcgttcccgaatatgttggtcataccgctggtttggttatcggtgcaggtggcacttctagagccgccctttacgccttgcacagtttaggttgcaaaaagatcttcataatcaacaggacaacttcgaaattgaagccattaatagagtcacttccatctgaattcaacattattggaatagagtccactaaatctatagaagagattaaggaacacgttggcgttgctgtcagctgtgtaccagccgacaaaccattagatgacgaacttttaagtaagctggagagattccttgtgaaaggtgcccatgctgcttttgtaccaaccttattggaagccgcatacaaaccaagcgttactcccgttatgacaatttcacaagacaaatatcaatggcacgttgtccctggatcacaaatgttagtacaccaaggtgtagctcagtttgaaaagtggacaggattcaagggccctttcaaggccatttttgatgccgttacgaaagagtag

SEQ ID NO: 4 - protein, 1588 aa, Saccharomyces cerevisiae
MVQLAKVPILGNDIIHVGYNIHDHLVETIIKHCPSSTYVICNDTNLSKVPYYQQLVLEFKASLPEGSRLLTYVVKPGETSKSRETKAQLEDYLLVEGCTRDTVMVAIGGGVIGDMIGFVASTFMRGVRVVQVPTSLLAMVDSSIGGKTAIDTPLGKNFIGAFWQPKFVLVDIKWLETLAKREFINGMAEVIKTACIWNADEFTRLESNASLFLNVVNGAKNVKVTNQLTNEIDEISNTDIEAMLDHTYKLVLESIKVKAEVVSSDERESSLRNLLNFGHSIGHAYEAILTPQALHGECVSIGMVKEAELSRYFGILSPTQVARLSKILVAYGLPVSPDEKWFKELTLHKKTPLDILLKKMSIDKKNEGSKKKVVILESIGKCYGDSAQFVSDEDLRFILTDETLVYPFKDIPADQQKVVIPPGSKSISNRALILAALGEGQCKIKNLLHSDDTKHMLTAVHELKGATISWEDNGETVVVEGHGGSTLSACADPLYLGNAGTASRFLTSLAALVNSTSSQKYIVLTGNARMQQRPIAPLVDSLRANGTKIEYLNNEGSLPIKVYTDSVFKGGRIELAATVSSQYVSSILMCAPYAEEPVTLALVGGKPISKLYVDMTIKMMEKFGINVETSTTEPYTYYIPKGHYINPSEYVIESDASSATYPLAFAAMTGTTVTVPNIGFESLQGDARFARDVLKPMGCKITQTATSTTVSGPPVGTLKPLKHVDMEPMTDAFLTACVVAAISHDSDPNSANTTTIEGIANQRVKECNRILAMATELAKFGVKTTELPDGIQVHGLNSIKDLKVPSDSSGPVGVCTYDDHRVAMSFSLLAGMVNSQNERDEVANPVRILERHCTGKTWPGWWDVLHSELGAKLDGAEPLECTSKKNSKKSVVIIGMRAAGKTTISKWCASALGYKLVDLDELFEQQHNNQSVKQFVVENGWEKFREEETRIFKEVIQNYGDDGYVFSTGGGIVESAESRKALKDFASSGGYVLHLHRDIEETIVFLQSDPSRPAYVEEIREVWNRREGWYKECSNFSFFAPHCSAEAEFQALRRSFSKYIATITGVREIEIPSGRSAFVCLTFDDLTEQTENLTPICYGCEAVEVRVDHLANYSADFVSKQLSILRKATDSIPIIFTVRTMKQGGNFPDEEFKTLRELYDIALKNGVEFLDLELTLPTDIQYEVINKRGNTKIIGSHHDFQGLYSWDDAEWENRFNQALTLDVDVVKFVGTAVNFEDNLRLEHFRDTHKNKPLIAVNMTSKGSISRVLNNVLTPVTSDLLPNSAAPGQLTVAQINKMYTSMGGIEPKELFVVGKPIGHSRSPILHNTGYEILGLPHKFDKFETESAQLVKEKLLDGNKNFGGAAVTIPLKLDIMQYMDELTDAAKVIGAVNTVIPLGNKKFKGDNTDWLGIRNALINNGVPEYVGHTAGLVIGAGGTSRAALYALHSLGCKKIFIINRTTSKLKPLIESLPSEFNIIGIESTKSIEEIKEHVGVAVSCVPADKPLDDELLSKLERFLVKGAHAAFVPTLLEAAYKPSVTPVMTISQDKYQWHVVPGSQMLVHQGVAQFEKWTGFKGPFKAIFDAVTKE

SEQ ID NO: 5 - DNA, 4767 bp, Artificial sequence
  Synthetic nucleic acid
atggtgcagttagccaaagtcccaattctaggaaatgatattatccacgttgggtataacattcatgaccatttggttgaaaccataattaaacattgtccttcttcgacatacgttatttgcaatgatacgaacttgagtaaagttccatactaccagcaattagtcctggaattcaaggcttctttgccagaaggctctcgtttacttacttatgttgttaaaccaggtgagacaagtaaaagtagagaaaccaaagcgcagctagaagattatcttttagtggaaggatgtactcgtgatacggttatggtagcgatcggtggtggtgttattggtgacatgattgggttcgttgcatctacatttatgagaggtgttcgtgttgtccaagtaccaacatccttattggcaatggtcgattcctccattggtggtaaaactgctattgacactcctctaggtaaaaactttattggtgcattttggcaaccaaaatttgtccttgtagatattaaatggctagaaacgttagccaagagagagtttatcaatgggatggcagaagttatcaagactgcttgtatttggaacgctgacgaatttactagattagaatcaaacgcttcgttgttcttaaatgttgttaatggggcaaaaaatgtcaaggttaccaatcaattgacaaacgagattgacgagatatcgaatacagatattgaagctatgttggatcatacatataagttagttcttgagagtattaaggtcaaagcggaagttgtctcttcggatgaacgtgaatccagtctaagaaaccttttgaacttcggacattctattggtcatgcttatgaagctatactaaccccacaagcattacatggtgaatgtgtgtccattggtatggttaaagaggcggaattatcccgttatttcggtattctctcccctacccaagttgcacgtctatccaagattttggttgcctacgggttgcctgtttcgcctgatgagaaatggtttaaagagctaaccttacataagaaaacaccattggatatcttattgaagaaaatgagtattgacaagaaaaacgagggttccaaaaagaaggtggtcattttagaaagtattggtaagtgctatggtgactccgctcaatttgttagcgatgaagacctgagatttattctaacagatgaaaccctcgtttaccccttcaaggacatccctgctgatcaacagaaagttgttatcccccctggttctaagtccatctccaatcgtgctttaattcttgctgccctcggtgaaggtcaatgtaaaatcaagaacttattacattctgatgatactaaacatatgttaaccgctgttcatgaattgaaaggtgctacgatatcatgggaagataatggtgagacggtagtggtggaaggacatggtggttccacattgtcagcttgtgctgaccccttatatctaggtaatgcaggtactgcatctagatttttgacttccttggctgccttggtcaattctacttcaagccaaaagtatatcgttttaactggtaacgcaagaatgcaacaaagaccaattgctcctttggtcgattctttgcgtgctaatggtactaaaattgagtacttgaataatgaaggttccctgccaatcaaagtttatactgattcggtattcaaaggtggtagaattgaattagctgctacagtttcttctcagtacgtatcctctatcttgatgtgtgccccatacgctgaagaacctgtaactttggctcttgttggtggtaagccaatctctaaattgtacgtcgatatgacaataaaaatgatggaaaaattcggtatcaatgttgaaacttctactacagaaccttacacttattatattccaaagggacattatattaacccatcagaatacgtcattgaaagtgatgcctcaagtgctacatacccattggccttcgccgcaatgactggtactaccgtaacggttccaaacattggttttgagtcgttacaaggtgatgccagatttgcaagagatgtcttgaaacctatgggttgtaaaataactcaaacggcaacttcaactactgtttcgggtcctcctgtaggtactttaaagccattaaaacatgttgatatggagccaatgactgatgcgttcttaactgcatgtgttgttgccgctatttcgcacgacagtgatccaaattctgcaaatacaaccaccattgaaggtattgcaaaccagcgtgtcaaagagtgtaacagaattttggccatggctacagagctcgccaaatttggcgtcaaaactacagaattaccagatggtattcaagtccatggtttaaactcgataaaagatttgaaggttccttccgactcttctggacctgtcggtgtatgcacatatgatgatcatcgtgtggccatgagtttctcgcttcttgcaggaatggtaaattctcaaaatgaacgtgacgaagttgctaatcctgtaagaatacttgaaagacattgtactggtaaaacctggcctggctggtgggatgtgttacattccgaactaggtgccaaattagatggtgcagaacctttagagtgcacatccaaaaagaactcaaagaaaagcgttgtcattattggcatgagagcagctggcaaaactactataagtaaatggtgcgcatccgctctgggttacaaattagttgacctagacgagctgtttgagcaacagcataacaatcaaagtgttaaacaatttgttgtggagaacggttgggagaagttccgtgaggaagaaacaagaattttcaaggaagttattcaaaattacggcgatgatggatatgttttctcaacaggtggcggtattgttgaaagcgctgagtctagaaaagccttaaaagattttgcctcatcaggtggatacgttttacacttacatagggatattgaggagacaattgtctttttacaaagtgatccttcaagacctgcctatgtggaagaaattcgtgaagtttggaacagaagggaggggtggtataaagaatgctcaaatttctctttctttgctcctcattgctccgcagaagctgagttccaagctctaagaagatcgtttagtaagtacattgcaaccattacaggtgtcagagaaatagaaattccaagcggaagatctgcctttgtgtgtttaacctttgatgacttaactgaacaaactgagaatttgactccaatctgttatggttgtgaggctgtagaggtcagagtagaccatttggctaattactctgctgatttcgtgagtaaacagttatctatattgcgtaaagccactgacagtattcctatcatttttactgtgcgaaccatgaagcaaggtggcaactttcctgatgaagagttcaaaaccttgagagagctatacgatattgccttgaagaatggtgttgaattccttgacttagaactaactttacctactgatatccaatatgaggttattaacaaaaggggcaacaccaagatcattggttcccatcatgacttccaaggattatactcctgggacgacgctgaatgggaaaacagattcaatcaagcgttaactcttgatgtggatgttgtaaaatttgtgggtacggctgttaatttcgaagataatttgagactggaacactttagggatacacacaagaataagcctttaattgcagttaatatgacttctaaaggtagcatttctcgtgttttgaataatgttttaacacctgtgacatcagatttattgcctaactccgctgcccctggccaattgacagtagcacaaattaacaagatgtatacatctatgggaggtatcgagcctaaggaactgtttgttgttggaaagccaattggccactctagatcgccaattttacataacactggctatgaaattttaggtttacctcacaagttcgataaatttgaaactgaatccgcacaattggtgaaagaaaaacttttggacggaaacaagaactttggcggtgctgcagtcacaattcctctgaaattagatataatgcagtacatggatgaattgactgatgctgctaaagttattggtgctgtaaacacagttataccattgggtaacaagaagtttaagggtgataataccgactggttaggtatccgtaatgccttaattaacaatggcgttcccgaatatgttggtcataccgctggtttggttatcggtgcaggtggcacttctagagccgccctttacgccttgcacagtttaggttgcaaaaagatcttcataatcaacaggacaacttcgaaattgaagccattaatagagtcacttccatctgaattcaacattattggaatagagtccactaaatctatagaagagattaaggaacacgttggcgttgctgtcagctgtgtaccagccgacaaaccattagatgacgaacttttaagtaagctggagagattccttgtgaaaggtgcccatgctgcttttgtaccaaccttattggaagccccatacaaaccaagcgttactcccgttatgacaatttcacaagacaaatatcaatggcacgttgtccctggatcacaaatgttagtacaccaaggtgtagctcagtttgaaaagtggacaggattcaagggccctttcaaggccatttttgatgccgttacgaaagagtag

SEQ ID NO: 6 - protein, 1588 aa, Artificial sequence
  Synthethic polypeptide
MVQLAKVPILGNDIIHVGYNIHDHLVETIIKHCPSSTYVICNDTNLSKVPYYQQLVLEFKASLPEGSRLLTYVVKPGETSKSRETKAQLEDYLLVEGCTRDTVMVAIGGGVIGDMIGFVASTFMRGVRVVQVPTSLLAMVDSSIGGKTAIDTPLGKNFIGAFWQPKFVLVDIKWLETLAKREFINGMAEVIKTACIWNADEFTRLESNASLFLNVVNGAKNVKVTNQLTNEIDEISNTDIEAMLDHTYKLVLESIKVKAEVVSSDERESSLRNLLNFGHSIGHAYEAILTPQALHGECVSIGMVKEAELSRYFGILSPTQVARLSKILVAYGLPVSPDEKWFKELTLHKKTPLDILLKKMSIDKKNEGSKKKVVILESIGKCYGDSAQFVSDEDLRFILTDETLVYPFKDIPADQQKVVIPPGSKSISNRALILAALGEGQCKIKNLLHSDDTKHMLTAVHELKGATISWEDNGETVVVEGHGGSTLSACADPLYLGNAGTASRFLTSLAALVNSTSSQKYIVLTGNARMQQRPIAPLVDSLRANGTKIEYLNNEGSLPIKVYTDSVFKGGRIELAATVSSQYVSSILMCAPYAEEPVTLALVGGKPISKLYVDMTIKMMEKFGINVETSTTEPYTYYIPKGHYINPSEYVIESDASSATYPLAFAAMTGTTVTVPNIGFESLQGDARFARDVLKPMGCKITQTATSTTVSGPPVGTLKPLKHVDMEPMTDAFLTACVVAAISHDSDPNSANTTTIEGIANQRVKECNRILAMATELAKFGVKTTELPDGIQVHGLNSIKDLKVPSDSSGPVGVCTYDDHRVAMSFSLLAGMVNSQNERDEVANPVRILERHCTGKTWPGWWDVLHSELGAKLDGAEPLECTSKKNSKKSVVIIGMRAAGKTTISKWCASALGYKLVDLDELFEQQHNNQSVKQFVVENGWEKFREEETRIFKEVIQNYGDDGYVFSTGGGIVESAESRKALKDFASSGGYVLHLHRDIEETIVFLQSDPSRPAYVEEIREVWNRREGWYKECSNFSFFAPHCSAEAEFQALRRSFSKYIATITGVREIEIPSGRSAFVCLTFDDLTEQTENLTPICYGCEAVEVRVDHLANYSADFVSKQLSILRKATDSIPIIFTVRTMKQGGNFPDEEFKTLRELYDIALKNGVEFLDLELTLPTDIQYEVINKRGNTKIIGSHHDFQGLYSWDDAEWENRFNQALTLDVDVVKFVGTAVNFEDNLRLEHFRDTHKNKPLIAVNMTSKGSISRVLNNVLTPVTSDLLPNSAAPGQLTVAQINKMYTSMGGIEPKELFVVGKPIGHSRSPILHNTGYEILGLPHKFDKFETESAQLVKEKLLDGNKNFGGAAVTIPLKLDIMQYMDELTDAAKVIGAVNTVIPLGNKKFKGDNTDWLGIRNALINNGVPEYVGHTAGLVIGAGGTSRAALYALHSLGCKKIFIINRTTSKLKPLIESLPSEFNIIGIESTKSIEEIKEHVGVAVSCVPADKPLDDELLSKLERFLVKGAHAAFVPTLLEAPYKPSVTPVMTISQDKYQWHVVPGSQMLVHQGVAQFEKWTGFKGPFKAIFDAVTKE

SEQ ID NO: 7 - DNA, 4767 bp, Artificial sequence
  Synthetic nucleic acid
atggtgcagttagccaaagtcccaattctaggaaatgatattatccacgttgggtataacattcatgaccatttggttgaaaccataattaaacattgtccttcttcgacatacgttatttgcaatgatacgaacttgagtaaagttccatactaccagcaattagtcctggaattcaaggcttctttgccagaaggctctcgtttacttacttatgttgttaaaccaggtgagacaagtaaaagtagagaaaccaaagcgcagctagaagattatcttttagtggaaggatgtactcgtgatacggttatggtagcgatcggtggtggtgttattggtgacatgattgggttcgttgcatctacatttatgagaggtgttcgtgttgtccaagtaccaacatccttattggcaatggtcgattcctccattggtggtaaaactgctattgacactcctctaggtaaaaactttattggtgcattttggcaaccaaaatttgtccttgtagatattaaatggctagaaacgttagccaagagagagtttatcaatgggatggcagaagttatcaagactgcttgtatttggaacgctgacgaatttactagattagaatcaaacgcttcgttgttcttaaatgttgttaatggggcaaaaaatgtcaaggttaccaatcaattgacaaacgagattgacgagatatcgaatacagatattgaagctatgttggatcatacatataagttagttcttgagagtattaaggtcaaagcggaagttgtctcttcggatgaacgtgaatccagtctaagaaaccttttgaacttcggacattctattggtcatgcttatgaagctatactaaccccacaagcattacatggtgaatgtgtgtccattggtatggttaaagaggcggaattatcccgttatttcggtattctctcccctacccaagttgcacgtctatccaagattttggttgcctacgggttgcctgtttcgcctgatgagaaatggtttaaagagctaaccttacataagaaaacaccattggatatcttattgaagaaaatgagtattgacaagaaaaacgagggttccaaaaagaaggtggtcattttagaaagtattggtaagtgctatggtgactccgctcaatttgttagcgatgaagacctgagatttattctaacagatgaaaccctcgtttaccccttcaaggacatccctgctgatcaacagaaagttgttatcccccctggttctaagtccatctccaatcgtgctttaattcttgctgccctcggtgaaggtcaatgtaaaatcaagaacttattacattctgatgatactaaacatatgttaaccgctgttcatgaattgaaaggtgctacgatatcatgggaagataatggtgagacggtagtggtggaaggacatggtggttccacattgtcagcttgtgctgaccccttatatctaggtaatgcaggtactgcatctagatttttgacttccttggctgccttggtcaattctacttcaagccaaaagtatatcgttttaactggtaacgcaagaatgcaacaaagaccaattgctcctttggtcgattctttgcgtgctaatggtactaaaattgagtacttgaataatgaaggttccctgccaatcaaagtttatactgattcggtattcaaaggtggtagaattgaattagctgctacagtttcttctcagtacgtatcctctatcttgatgtgtgccccatacgctgaagaacctgtaactttggctcttgttggtggtaagccaatctctaaattgtacgtcgatatgacaataaaaatgatggaaaaattcggtatcaatgttgaaacttctactacagaaccttacacttattatattccaaagggacattatattaacccatcagaatacgtcattgaaagtgatgcctcaagtgctacatacccattggccttcgccgcaatgactggtactaccgtaacggttccaaacattggttttgagtcgttacaaggtgatgccagatttgcaagagatgtcttgaaacctatgggttgtaaaataactcaaacggcaacttcaactactgtttcgggtcctcctgtaggtactttaaagccattaaaacatgttgatatggagccaatgactgatgcgttcttaactgcatgtgttgttgccgctatttcgcacgacagtgatccaaattctgcaaatacaaccaccattgaaggtattgcaaaccagcgtgtcaaagagtgtaacagaattttggccatggctacagagctcgccaaatttggcgtcaaaactacagaattaccagatggtattcaagtccatggtttaaactcgataaaagatttgaaggttccttccgactcttctggacctgtcggtgtatgcacatatgatgatcatcgtgtggccatgagtttctcgcttcttgcaggaatggtaaattctcaaaatgaacgtgacgaagttgctaatcctgtaagaatacttgaaagacattgtactggtaaaacctggcctggctggtgggatgtgttacattccgaactaggtgccaaattagatggtgcagaacctttagagtgcacatccaaaaagaactcaaagaaaagcgttgtcattattggcatgagagcagctggcaaaactactataagtaaatggtgcgcatccgctctgggttacaaattagttgacctagacgagctgtttgagcaacagcataacaatcaaagtgttaaacaatttgttgtggagaacggttgggagaagttccgtgaggaagaaacaagaattttcaaggaagttattcaaaattacggcgatgatggatatgttttctcaacaggtggcggtattgttgaaagcgctgagtctagaaaagccttaaaagattttgcctcatcaggtggatacgttttacacttacatagggatattgaggagacaattgtctttttacaaagtgatccttcaagacctgcctatgtggaagaaattcgtgaagtttggaacagaagggaggggtggtataaagaatgctcaaatttctctttctttgctcctcattgctccgcagaagctgagttccaagctctaagaagatcgtttagtaagtacattgcaaccattacaggtgtcagagaaatagaaattccaagcggaagatctgcctttgtgtgtttaacctttgatgacttaactgaacaaactgagaatttgactccaatctgttatggttgtgaggctgtagaggtcagagtagaccatttggctaattactctgctgatttcgtgagtaaacagttatctatattgcgtaaagccactgacagtattcctatcatttttactgtgcgaaccatgaagcaaggtggcaactttcctgatgaagagttcaaaaccttgagagagctatacgatattgccttgaagaatggtgttgaattccttgacttagaactaactttacctactgatatccaatatgaggttattaacaaaaggggcaacaccaagatcattggttcccatcatgacttccaaggattatactcctgggacgacgctgaatgggaaaacagattcaatcaagcgttaactcttgatgtggatgttgtaaaatttgtgggtacggctgttaatttcgaagataatttgagactggaacactttagggatacacacaagaataagcctttaattgcagttaatatgacttctaaaggtagcatttctcgtgttttgaataatgttttaacacctgtgacatcagatttattgcctaactccgctgcccctggccaattgacagtagcacaaattaacaagatgtatacatctatgggaggtatcgagcctaaggaactgtttgttgttggaaagccaattggccactctagatcgccaattttacataacactggctatgaaattttaggtttacctcacaagttcgataaatttgaaactgaatccgcacaattggtgaaagaaaaacttttggacggaaacaagaactttggcggtgctgcagtcacaattcctctgaaattagatataatgcagtacatggatgaattgactgatgctgctaaagttattggtgctgtaaacacagttataccattgggtaacaagaagtttaagggtgataataccgactggttaggtatccgtaatgccttaattaacaatggcgttcccgaatatgttggtcataccgctggtttggttatcggtgcaggtggcacttctagagccgccctttacgccttgcacagtttaggttgcaaaaagatcttcataatcaacaggacaacttcgaaattgaagccattaatagagtcacttccatctgaattcaacattattggaatagagtccactaaatctatagaagagattaaggaacacgttggcgttgctgtcagctgtgtaaaagccgacaaaccattagatgacgaacttttaagtaagctggagagattccttgtgaaaggtgcccatgctgcttttgtaccaaccttattggaagccgcatacaaaccaagcgttactcccgttatgacaatttcacaagacaaatatcaatggcacgttgtccctggatcacaaatgttagtacaccaaggtgtagctcagtttgaaaagtggacaggattcaagggccctttcaaggccatttttgatgccgttacgaaagagtag

SEQ ID NO: 8 - protein, 1588 aa, Artificial sequence
  Synthetic polypeptide
MVQLAKVPILGNDIIHVGYNIHDHLVETIIKHCPSSTYVICNDTNLSKVPYYQQLVLEFKASLPEGSRLLTYVVKPGETSKSRETKAQLEDYLLVEGCTRDTVMVAIGGGVIGDMIGFVASTFMRGVRVVQVPTSLLAMVDSSIGGKTAIDTPLGKNFIGAFWQPKFVLVDIKWLETLAKREFINGMAEVIKTACIWNADEFTRLESNASLFLNVVNGAKNVKVTNQLTNEIDEISNTDIEAMLDHTYKLVLESIKVKAEVVSSDERESSLRNLLNFGHSIGHAYEAILTPQALHGECVSIGMVKEAELSRYFGILSPTQVARLSKILVAYGLPVSPDEKWFKELTLHKKTPLDILLKKMSIDKKNEGSKKKVVILESIGKCYGDSAQFVSDEDLRFILTDETLVYPFKDIPADQQKVVIPPGSKSISNRALILAALGEGQCKIKNLLHSDDTKHMLTAVHELKGATISWEDNGETVVVEGHGGSTLSACADPLYLGNAGTASRFLTSLAALVNSTSSQKYIVLTGNARMQQRPIAPLVDSLRANGTKIEYLNNEGSLPIKVYTDSVFKGGRIELAATVSSQYVSSILMCAPYAEEPVTLALVGGKPISKLYVDMTIKMMEKFGINVETSTTEPYTYYIPKGHYINPSEYVIESDASSATYPLAFAAMTGTTVTVPNIGFESLQGDARFARDVLKPMGCKITQTATSTTVSGPPVGTLKPLKHVDMEPMTDAFLTACVVAAISHDSDPNSANTTTIEGIANQRVKECNRILAMATELAKFGVKTTELPDGIQVHGLNSIKDLKVPSDSSGPVGVCTYDDHRVAMSFSLLAGMVNSQNERDEVANPVRILERHCTGKTWPGWWDVLHSELGAKLDGAEPLECTSKKNSKKSVVIIGMRAAGKTTISKWCASALGYKLVDLDELFEQQHNNQSVKQFVVENGWEKFREEETRIFKEVIQNYGDDGYVFSTGGGIVESAESRKALKDFASSGGYVLHLHRDIEETIVFLQSDPSRPAYVEEIREVWNRREGWYKECSNFSFFAPHCSAEAEFQALRRSFSKYIATITGVREIEIPSGRSAFVCLTFDDLTEQTENLTPICYGCEAVEVRVDHLANYSADFVSKQLSILRKATDSIPIIFTVRTMKQGGNFPDEEFKTLRELYDIALKNGVEFLDLELTLPTDIQYEVINKRGNTKIIGSHHDFQGLYSWDDAEWENRFNQALTLDVDVVKFVGTAVNFEDNLRLEHFRDTHKNKPLIAVNMTSKGSISRVLNNVLTPVTSDLLPNSAAPGQLTVAQINKMYTSMGGIEPKELFVVGKPIGHSRSPILHNTGYEILGLPHKFDKFETESAQLVKEKLLDGNKNFGGAAVTIPLKLDIMQYMDELTDAAKVIGAVNTVIPLGNKKFKGDNTDWLGIRNALINNGVPEYVGHTAGLVIGAGGTSRAALYALHSLGCKKIFIINRTTSKLKPLIESLPSEFNIIGIESTKSIEEIKEHVGVAVSCVKADKPLDDELLSKLERFLVKGAHAAFVPTLLEAAYKPSVTPVMTISQDKYQWHVVPGSQMLVHQGVAQFEKWTGFKGPFKAIFDAVTKE

SEQ ID NO: 9 - DNA, 4767 bp, Artificial sequence
  Synthetic nucleic acid
atggtgcagttagccaaagtcccaattctaggaaatgatattatccacgttgggtataacattcatgaccatttggttgaaaccataattaaacattgtccttcttcgacatacgttatttgcaatgatacgaacttgagtaaagttccatactaccagcaattagtcctggaattcaaggcttctttgccagaaggctctcgtttacttacttatgttgttaaaccaggtgagacaagtaaaagtagagaaaccaaagcgcagctagaagattatcttttagtggaaggatgtactcgtgatacggttatggtagcgatcggtggtggtgttattggtgacatgattgggttcgttgcatctacatttatgagaggtgttcgtgttgtccaagtaccaacatccttattggcaatggtcgattcctccattggtggtaaaactgctattgacactcctctaggtaaaaactttattggtgcattttggcaaccaaaatttgtccttgtagatattaaatggctagaaacgttagccaagagagagtttatcaatgggatggcagaagttatcaagactgcttgtatttggaacgctgacgaatttactagattagaatcaaacgcttcgttgttcttaaatgttgttaatggggcaaaaaatgtcaaggttaccaatcaattgacaaacgagattgacgagatatcgaatacagatattgaagctatgttggatcatacatataagttagttcttgagagtattaaggtcaaagcggaagttgtctcttcggatgaacgtgaatccagtctaagaaaccttttgaacttcggacattctattggtcatgcttatgaagctatactaaccccacaagcattacatggtgaatgtgtgtccattggtatggttaaagaggcggaattatcccgttatttcggtattctctcccctacccaagttgcacgtctatccaagattttggttgcctacgggttgcctgtttcgcctgatgagaaatggtttaaagagctaaccttacataagaaaacaccattggatatcttattgaagaaaatgagtattgacaagaaaaacgagggttccaaaaagaaggtggtcattttagaaagtattggtaagtgctatggtgactccgctcaatttgttagcgatgaagacctgagatttattctaacagatgaaaccctcgtttaccccttcaaggacatccctgctgatcaacagaaagttgttatcccccctggttctaagtccatctccaatcgtgctttaattcttgctgccctcggtgaaggtcaatgtaaaatcaagaacttattacattctgatgatactaaacatatgttaaccgctgttcatgaattgaaaggtgctacgatatcatgggaagataatggtgagacggtagtggtggaaggacatggtggttccacattgtcagcttgtgctgaccccttatatctaggtaatgcaggtactgcatctagatttttgacttccttggctgccttggtcaattctacttcaagccaaaagtatatcgttttaactggtaacgcaagaatgcaacaaagaccaattgctcctttggtcgattctttgcgtgctaatggtactaaaattgagtacttgaataatgaaggttccctgccaatcaaagtttatactgattcggtattcaaaggtggtagaattgaattagctgctacagtttcttctcagtacgtatcctctatcttgatgtgtgccccatacgctgaagaacctgtaactttggctcttgttggtggtaagccaatctctaaattgtacgtcgatatgacaataaaaatgatggaaaaattcggtatcaatgttgaaacttctactacagaaccttacacttattatattccaaagggacattatattaacccatcagaatacgtcattgaaagtgatgcctcaagtgctacatacccattggccttcgccgcaatgactggtactaccgtaacggttccaaacattggttttgagtcgttacaaggtgatgccagatttgcaagagatgtcttgaaacctatgggttgtaaaataactcaaacggcaacttcaactactgtttcgggtcctcctgtaggtactttaaagccattaaaacatgttgatatggagccaatgactgatgcgttcttaactgcatgtgttgttgccgctatttcgcacgacagtgatccaaattctgcaaatacaaccaccattgaaggtattgcaaaccagcgtgtcaaagagtgtaacagaattttggccatggctacagagctcgccaaatttggcgtcaaaactacagaattaccagatggtattcaagtccatggtttaaactcgataaaagatttgaaggttccttccgactcttctggacctgtcggtgtatgcacatatgatgatcatcgtgtggccatgagtttctcgcttcttgcaggaatggtaaattctcaaaatgaacgtgacgaagttgctaatcctgtaagaatacttgaaagacattgtactggtaaaacctggcctggctggtgggatgtgttacattccgaactaggtgccaaattagatggtgcagaacctttagagtgcacatccaaaaagaactcaaagaaaagcgttgtcattattggcatgagagcagctggcaaaactactataagtaaatggtgcgcatccgctctgggttacaaattagttgacctagacgagctgtttgagcaacagcataacaatcaaagtgttaaacaatttgttgtggagaacggttgggagaagttccgtgaggaagaaacaagaattttcaaggaagttattcaaaattacggcgatgatggatatgttttctcaacaggtggcggtattgttgaaagcgctgagtctagaaaagccttaaaagattttgcctcatcaggtggatacgttttacacttacatagggatattgaggagacaattgtctttttacaaagtgatccttcaagacctgcctatgtggaagaaattcgtgaagtttggaacagaagggaggggtggtataaagaatgctcaaatttctctttctttgctcctcattgctccgcagaagctgagttccaagctctaagaagatcgtttagtaagtacattgcaaccattacaggtgtcagagaaatagaaattccaagcggaagatctgcctttgtgtgtttaacctttgatgacttaactgaacaaactgagaatttgactccaatctgttatggttgtgaggctgtagaggtcagagtagaccatttggctaattactctgctgatttcgtgagtaaacagttatctatattgcgtaaagccactgacagtattcctatcatttttactgtgcgaaccatgaagcaaggtggcaactttcctgatgaagagttcaaaaccttgagagagctatacgatattgccttgaagaatggtgttgaattccttgacttagaactaactttacctactgatatccaatatgaggttattaacaaaaggggcaacaccaagatcattggttcccatcatgacttccaaggattatactcctgggacgacgctgaatgggaaaacagattcaatcaagcgttaactcttgatgtggatgttgtaaaatttgtgggtacggctgttaatttcgaagataatttgagactggaacactttagggatacacacaagaataagcctttaattgcagttaatatgacttctaaaggtagcatttctcgtgttttgaataatgttttaacacctgtgacatcagatttattgcctaactccgctgcccctggccaattgacagtagcacaaattaacaagatgtatacatctatgggaggtatcgagcctaaggaactgtttgttgttggaaagccaattggccactctagatcgccaattttacataacactggctatgaaattttaggtttacctcacaagttcgataaatttgaaactgaatccgcacaattggtgaaagaaaaacttttggacggaaacaagaactttggcggtgctgcagtcacaattcctctgaaattagatataatgcagtacatggatgaattgactgatgctgctaaagttattggtgctgtaaacacagttataccattgggtaacaagaagtttaagggtgataataccgactggttaggtatccgtaatgccttaattaacaatggcgttcccgaatatgttggtcataccgctggtttggttatcggtgcaggtggcacttctagagccgccctttacgccttgcacagtttaggttgcaaaaagatcttcataatcaactggacaacttcgaaattgaagccattaatagagtcacttccatctgaattcaacattattggaatagagtccactaaatctatagaagagattaaggaacacgttggcgttgctgtcagctgtgtaccagccgacaaaccattagatgacgaacttttaagtaagctggagagattccttgtgaaaggtgcccatgctgcttttgtaccaaccttattggaagccgcatacaaaccaagcgttactcccgttatgacaatttcacaagacaaatatcaatggcacgttgtccctggatcacaaatgttagtacaccaaggtgtagctcagtttgaaaagtggacaggattcaagggccctttcaaggccatttttgatgccgttacgaaagagtag

SEQ ID NO: 10 - protein, 1588 aa, Artificial sequence
  Synthetic polypeptide
MVQLAKVPILGNDIIHVGYNIHDHLVETIIKHCPSSTYVICNDTNLSKVPYYQQLVLEFKASLPEGSRLLTYVVKPGETSKSRETKAQLEDYLLVEGCTRDTVMVAIGGGVIGDMIGFVASTFMRGVRVVQVPTSLLAMVDSSIGGKTAIDTPLGKNFIGAFWQPKFVLVDIKWLETLAKREFINGMAEVIKTACIWNADEFTRLESNASLFLNVVNGAKNVKVTNQLTNEIDEISNTDIEAMLDHTYKLVLESIKVKAEVVSSDERESSLRNLLNFGHSIGHAYEAILTPQALHGECVSIGMVKEAELSRYFGILSPTQVARLSKILVAYGLPVSPDEKWFKELTLHKKTPLDILLKKMSIDKKNEGSKKKVVILESIGKCYGDSAQFVSDEDLRFILTDETLVYPFKDIPADQQKVVIPPGSKSISNRALILAALGEGQCKIKNLLHSDDTKHMLTAVHELKGATISWEDNGETVVVEGHGGSTLSACADPLYLGNAGTASRFLTSLAALVNSTSSQKYIVLTGNARMQQRPIAPLVDSLRANGTKIEYLNNEGSLPIKVYTDSVFKGGRIELAATVSSQYVSSILMCAPYAEEPVTLALVGGKPISKLYVDMTIKMMEKFGINVETSTTEPYTYYIPKGHYINPSEYVIESDASSATYPLAFAAMTGTTVTVPNIGFESLQGDARFARDVLKPMGCKITQTATSTTVSGPPVGTLKPLKHVDMEPMTDAFLTACVVAAISHDSDPNSANTTTIEGIANQRVKECNRILAMATELAKFGVKTTELPDGIQVHGLNSIKDLKVPSDSSGPVGVCTYDDHRVAMSFSLLAGMVNSQNERDEVANPVRILERHCTGKTWPGWWDVLHSELGAKLDGAEPLECTSKKNSKKSVVIIGMRAAGKTTISKWCASALGYKLVDLDELFEQQHNNQSVKQFVVENGWEKFREEETRIFKEVIQNYGDDGYVFSTGGGIVESAESRKALKDFASSGGYVLHLHRDIEETIVFLQSDPSRPAYVEEIREVWNRREGWYKECSNFSFFAPHCSAEAEFQALRRSFSKYIATITGVREIEIPSGRSAFVCLTFDDLTEQTENLTPICYGCEAVEVRVDHLANYSADFVSKQLSILRKATDSIPIIFTVRTMKQGGNFPDEEFKTLRELYDIALKNGVEFLDLELTLPTDIQYEVINKRGNTKIIGSHHDFQGLYSWDDAEWENRFNQALTLDVDVVKFVGTAVNFEDNLRLEHFRDTHKNKPLIAVNMTSKGSISRVLNNVLTPVTSDLLPNSAAPGQLTVAQINKMYTSMGGIEPKELFVVGKPIGHSRSPILHNTGYEILGLPHKFDKFETESAQLVKEKLLDGNKNFGGAAVTIPLKLDIMQYMDELTDAAKVIGAVNTVIPLGNKKFKGDNTDWLGIRNALINNGVPEYVGHTAGLVIGAGGTSRAALYALHSLGCKKIFIINWTTSKLKPLIESLPSEFNIIGIESTKSIEEIKEHVGVAVSCVPADKPLDDELLSKLERFLVKGAHAAFVPTLLEAAYKPSVTPVMTISQDKYQWHVVPGSQMLVHQGVAQFEKWTGFKGPFKAIFDAVTKE

SEQ ID NO: 11 - DNA, 4767 bp, Artificial sequence
  Synthetic nucleic acid
atggtgcagttagccaaagtcccaattctaggaaatgatattatccacgttgggtataacattcatgaccatttggttgaaaccataattaaacattgtccttcttcgacatacgttatttgcaatgatacgaacttgagtaaagttccatactaccagcaattagtcctggaattcaaggcttctttgccagaaggctctcgtttacttacttatgttgttaaaccaggtgagacaagtaaaagtagagaaaccaaagcgcagctagaagattatcttttagtggaaggatgtactcgtgatacggttatggtagcgatcggtggtggtgttattggtgacatgattgggttcgttgcatctacatttatgagaggtgttcgtgttgtccaagtaccaacatccttattggcaatggtcgattcctccattggtggtaaaactgctattgacactcctctaggtaaaaactttattggtgcattttggcaaccaaaatttgtccttgtagatattaaatggctagaaacgttagccaagagagagtttatcaatgggatggcagaagttatcaagactgcttgtatttggaacgctgacgaatttactagattagaatcaaacgcttcgttgttcttaaatgttgttaatggggcaaaaaatgtcaaggttaccaatcaattgacaaacgagattgacgagatatcgaatacagatattgaagctatgttggatcatacatataagttagttcttgagagtattaaggtcaaagcggaagttgtctcttcggatgaacgtgaatccagtctaagaaaccttttgaacttcggacattctattggtcatgcttatgaagctatactaaccccacaagcattacatggtgaatgtgtgtccattggtatggttaaagaggcggaattatcccgttatttcggtattctctcccctacccaagttgcacgtctatccaagattttggttgcctacgggttgcctgtttcgcctgatgagaaatggtttaaagagctaaccttacataagaaaacaccattggatatcttattgaagaaaatgagtattgacaagaaaaacgagggttccaaaaagaaggtggtcattttagaaagtattggtaagtgctatggtgactccgctcaatttgttagcgatgaagacctgagatttattctaacagatgaaaccctcgtttaccccttcaaggacatccctgctgatcaacagaaagttgttatcccccctggttctaagtccatctccaatcgtgctttaattcttgctgccctcggtgaaggtcaatgtaaaatcaagaacttattacattctgatgatactaaacatatgttaaccgctgttcatgaattgaaaggtgctacgatatcatgggaagataatggtgagacggtagtggtggaaggacatggtggttccacattgtcagcttgtgctgaccccttatatctaggtaatgcaggtactgcatctagatttttgacttccttggctgccttggtcaattctacttcaagccaaaagtatatcgttttaactggtaacgcaagaatgcaacaaagaccaattgctcctttggtcgattctttgcgtgctaatggtactaaaattgagtacttgaataatgaaggttccctgccaatcaaagtttatactgattcggtattcaaaggtggtagaattgaattagctgctacagtttcttctcagtacgtatcctctatcttgatgtgtgccccatacgctgaagaacctgtaactttggctcttgttggtggtaagccaatctctaaattgtacgtcgatatgacaataaaaatgatggaaaaattcggtatcaatgttgaaacttctactacagaaccttacacttattatattccaaagggacattatattaacccatcagaatacgtcattgaaagtgatgcctcaagtgctacatacccattggccttcgccgcaatgactggtactaccgtaacggttccaaacattggttttgagtcgttacaaggtgatgccagatttgcaagagatgtcttgaaacctatgggttgtaaaataactcaaacggcaacttcaactactgtttcgggtcctcctgtaggtactttaaagccattaaaacatgttgatatggagccaatgactgatgcgttcttaactgcatgtgttgttgccgctatttcgcacgacagtgatccaaattctgcaaatacaaccaccattgaaggtattgcaaaccagcgtgtcaaagagtgtaacagaattttggccatggctacagagctcgccaaatttggcgtcaaaactacagaattaccagatggtattcaagtccatggtttaaactcgataaaagatttgaaggttccttccgactcttctggacctgtcggtgtatgcacatatgatgatcatcgtgtggccatgagtttctcgcttcttgcaggaatggtaaattctcaaaatgaacgtgacgaagttgctaatcctgtaagaatacttgaaagacattgtactggtaaaacctggcctggctggtgggatgtgttacattccgaactaggtgccaaattagatggtgcagaacctttagagtgcacatccaaaaagaactcaaagaaaagcgttgtcattattggcatgagagcagctggcaaaactactataagtaaatggtgcgcatccgctctgggttacaaattagttgacctagacgagctgtttgagcaacagcataacaatcaaagtgttaaacaatttgttgtggagaacggttgggagaagttccgtgaggaagaaacaagaattttcaaggaagttattcaaaattacggcgatgatggatatgttttctcaacaggtggcggtattgttgaaagcgctgagtctagaaaagccttaaaagattttgcctcatcaggtggatacgttttacacttacatagggatattgaggagacaattgtctttttacaaagtgatccttcaagacctgcctatgtggaagaaattcgtgaagtttggaacagaagggaggggtggtataaagaatgctcaaatttctctttctttgctcctcattgctccgcagaagctgagttccaagctctaagaagatcgtttagtaagtacattgcaaccattacaggtgtcagagaaatagaaattccaagcggaagatctgcctttgtgtgtttaacctttgatgacttaactgaacaaactgagaatttgactccaatctgttatggttgtgaggctgtagaggtcagagtagaccatttggctaattactctgctgatttcgtgagtaaacagttatctatattgcgtaaagccactgacagtattcctatcatttttactgtgcgaaccatgaagcaaggtggcaactttcctgatgaagagttcaaaaccttgagagagctatacgatattgccttgaagaatggtgttgaattccttgacttagaactaactttacctactgatatccaatatgaggttattaacaaaaggggcaacaccaagatcattggttcccatcatgacttccaaggattatactcctgggacgacgctgaatgggaaaacagattcaatcaagcgttaactcttgatgtggatgttgtaaaatttgtgggtacggctgttaatttcgaagataatttgagactggaacactttagggatacacacaagaataagcctttaattgcagttaatatgacttctaaaggtagcatttctcgtgttttgaataatgttttaacacctgtgacatcagatttattgcctaactccgctgcccctggccaattgacagtagcacaaattaacaagatgtatacatctatgggaggtatcgagcctaaggaactgtttgttgttggaaagccaattggccactctagatcgccaattttacataacactggctatgaaattttaggtttacctcacaagttcgataaatttgaaactgaatccgcacaattgggaaaagaaaaacttttggacggaaacaagaactttggcggtgctgcagtcacaattcctctgaaattagatataatgcagtacatggatgaattgactgatgctgctaaagttattggtgctgtaaacacagttataccattgggtaacaagaagtttaagggtgataataccgactggttaggtatccgtaatgccttaattaacaatggcgttcccgaatatgttggtcataccgctggtttggttatcggtgcaggtggcacttctagagccgccctttacgccttgcacagtttaggttgcaaaaagatcttcataatcaacaggacaacttcgaaattgaagccattaatagagtcacttccatctgaattcaacattattggaatagagtccactaaatctatagaagagattaaggaacacgttggcgttgctgtcagctgtgtaccagccgacaaaccattagatgacgaacttttaagtaagctggagagattccttgtgaaaggtgcccatgctgcttttgtaccaaccttattggaagccgcatacaaaccaagcgttactcccgttatgacaatttcacaagacaaatatcaatggcacgttgtccctggatcacaaatgttagtacaccaaggtgtagctcagtttgaaaagtggacaggattcaagggccctttcaaggccatttttgatgccgttacgaaagagtag

SEQ ID NO: 12 - protein, 1588 aa, Artificial sequence
  Synthetic polypeptide
MVQLAKVPILGNDIIHVGYNIHDHLVETIIKHCPSSTYVICNDTNLSKVPYYQQLVLEFKASLPEGSRLLTYVVKPGETSKSRETKAQLEDYLLVEGCTRDTVMVAIGGGVIGDMIGFVASTFMRGVRVVQVPTSLLAMVDSSIGGKTAIDTPLGKNFIGAFWQPKFVLVDIKWLETLAKREFINGMAEVIKTACIWNADEFTRLESNASLFLNVVNGAKNVKVTNQLTNEIDEISNTDIEAMLDHTYKLVLESIKVKAEVVSSDERESSLRNLLNFGHSIGHAYEAILTPQALHGECVSIGMVKEAELSRYFGILSPTQVARLSKILVAYGLPVSPDEKWFKELTLHKKTPLDILLKKMSIDKKNEGSKKKVVILESIGKCYGDSAQFVSDEDLRFILTDETLVYPFKDIPADQQKVVIPPGSKSISNRALILAALGEGQCKIKNLLHSDDTKHMLTAVHELKGATISWEDNGETVVVEGHGGSTLSACADPLYLGNAGTASRFLTSLAALVNSTSSQKYIVLTGNARMQQRPIAPLVDSLRANGTKIEYLNNEGSLPIKVYTDSVFKGGRIELAATVSSQYVSSILMCAPYAEEPVTLALVGGKPISKLYVDMTIKMMEKFGINVETSTTEPYTYYIPKGHYINPSEYVIESDASSATYPLAFAAMTGTTVTVPNIGFESLQGDARFARDVLKPMGCKITQTATSTTVSGPPVGTLKPLKHVDMEPMTDAFLTACVVAAISHDSDPNSANTTTIEGIANQRVKECNRILAMATELAKFGVKTTELPDGIQVHGLNSIKDLKVPSDSSGPVGVCTYDDHRVAMSFSLLAGMVNSQNERDEVANPVRILERHCTGKTWPGWWDVLHSELGAKLDGAEPLECTSKKNSKKSVVIIGMRAAGKTTISKWCASALGYKLVDLDELFEQQHNNQSVKQFVVENGWEKFREEETRIFKEVIQNYGDDGYVFSTGGGIVESAESRKALKDFASSGGYVLHLHRDIEETIVFLQSDPSRPAYVEEIREVWNRREGWYKECSNFSFFAPHCSAEAEFQALRRSFSKYIATITGVREIEIPSGRSAFVCLTFDDLTEQTENLTPICYGCEAVEVRVDHLANYSADFVSKQLSILRKATDSIPIIFTVRTMKQGGNFPDEEFKTLRELYDIALKNGVEFLDLELTLPTDIQYEVINKRGNTKIIGSHHDFQGLYSWDDAEWENRFNQALTLDVDVVKFVGTAVNFEDNLRLEHFRDTHKNKPLIAVNMTSKGSISRVLNNVLTPVTSDLLPNSAAPGQLTVAQINKMYTSMGGIEPKELFVVGKPIGHSRSPILHNTGYEILGLPHKFDKFETESAQLGKEKLLDGNKNFGGAAVTIPLKLDIMQYMDELTDAAKVIGAVNTVIPLGNKKFKGDNTDWLGIRNALINNGVPEYVGHTAGLVIGAGGTSRAALYALHSLGCKKIFIINRTTSKLKPLIESLPSEFNIIGIESTKSIEEIKEHVGVAVSCVPADKPLDDELLSKLERFLVKGAHAAFVPTLLEAAYKPSVTPVMTISQDKYQWHVVPGSQMLVHQGVAQFEKWTGFKGPFKAIFDAVTKE

SEQ ID NO: 13 - DNA, 4767 bp, Artificial sequence
  Synthetic nucleic acid
atggtgcagttagccaaagtcccaattctaggaaatgatattatccacgttgggtataacattcatgaccatttggttgaaaccataattaaacattgtccttcttcgacatacgttatttgcaatgatacgaacttgagtaaagttccatactaccagcaattagtcctggaattcaaggcttctttgccagaaggctctcgtttacttacttatgttgttaaaccaggtgagacaagtaaaagtagagaaaccaaagcgcagctagaagattatcttttagtggaaggatgtactcgtgatacggttatggtagcgatcggtggtggtgttattggtgacatgattgggttcgttgcatctacatttatgagaggtgttcgtgttgtccaagtaccaacatccttattggcaatggtcgattcctccattggtggtaaaactgctattgacactcctctaggtaaaaactttattggtgcattttggcaaccaaaatttgtccttgtagatattaaatggctagaaacgttagccaagagagagtttatcaatgggatggcagaagttatcaagactgcttgtatttggaacgctgacgaatttactagattagaatcaaacgcttcgttgttcttaaatgttgttaatggggcaaaaaatgtcaaggttaccaatcaattgacaaacgagattgacgagatatcgaatacagatattgaagctatgttggatcatacatataagttagttcttgagagtattaaggtcaaagcggaagttgtctcttcggatgaacgtgaatccagtctaagaaaccttttgaacttcggacattctattggtcatgcttatgaagctatactaaccccacaagcattacatggtgaatgtgtgtccattggtatggttaaagaggcggaattatcccgttatttcggtattctctcccctacccaagttgcacgtctatccaagattttggttgcctacgggttgcctgtttcgcctgatgagaaatggtttaaagagctaaccttacataagaaaacaccattggatatcttattgaagaaaatgagtattgacaagaaaaacgagggttccaaaaagaaggtggtcattttagaaagtattggtaagtgctatggtgactccgctcaatttgttagcgatgaagacctgagatttattctaacagatgaaaccctcgtttaccccttcaaggacatccctgctgatcaacagaaagttgttatcccccctggttctaagtccatctccaatcgtgctttaattcttgctgccctcggtgaaggtcaatgtaaaatcaagaacttattacattctgatgatactaaacatatgttaaccgctgttcatgaattgaaaggtgctacgatatcatgggaagataatggtgagacggtagtggtggaaggacatggtggttccacattgtcagcttgtgctgaccccttatatctaggtaatgcaggtactgcatctagatttttgacttccttggctgccttggtcaattctacttcaagccaaaagtatatcgttttaactggtaacgcaagaatgcaacaaagaccaattgctcctttggtcgattctttgcgtgctaatggtactaaaattgagtacttgaataatgaaggttccctgccaatcaaagtttatactgattcggtattcaaaggtggtagaattgaattagctgctacagtttcttctcagtacgtatcctctatcttgatgtgtgccccatacgctgaagaacctgtaactttggctcttgttggtggtaagccaatctctaaattgtacgtcgatatgacaataaaaatgatggaaaaattcggtatcaatgttgaaacttctactacagaaccttacacttattatattccaaagggacattatattaacccatcagaatacgtcattgaaagtgatgcctcaagtgctacatacccattggccttcgccgcaatgactggtactaccgtaacggttccaaacattggttttgagtcgttacaaggtgatgccagatttgcaagagatgtcttgaaacctatgggttgtaaaataactcaaacggcaacttcaactactgtttcgggtcctcctgtaggtactttaaagccattaaaacatgttgatatggagccaatgactgatgcgttcttaactgcatgtgttgttgccgctatttcgcacgacagtgatccaaattctgcaaatacaaccaccattgaaggtattgcaaaccagcgtgtcaaagagtgtaacagaattttggccatggctacagagctcgccaaatttggcgtcaaaactacagaattaccagatggtattcaagtccatggtttaaactcgataaaagatttgaaggttccttccgactcttctggacctgtcggtgtatgcacatatgatgatcatcgtgtggccatgagtttctcgcttcttgcaggaatggtaaattctcaaaatgaacgtgacgaagttgctaatcctgtaagaatacttgaaagacattgtactggtaaaacctggcctggctggtgggatgtgttacattccgaactaggtgccaaattagatggtgcagaacctttagagtgcacatccaaaaagaactcaaagaaaagcgttgtcattattggcatgagagcagctggcaaaactactataagtaaatggtgcgcatccgctctgggttacaaattagttgacctagacgagctgtttgagcaacagcataacaatcaaagtgttaaacaatttgttgtggagaacggttgggagaagttccgtgaggaagaaacaagaattttcaaggaagttattcaaaattacggcgatgatggatatgttttctcaacaggtggcggtattgttgaaagcgctgagtctagaaaagccttaaaagattttgcctcatcaggtggatacgttttacacttacatagggatattgaggagacaattgtctttttacaaagtgatccttcaagacctgcctatgtggaagaaattcgtgaagtttggaacagaagggaggggtggtataaagaatgctcaaatttctctttctttgctcctcattgctccgcagaagctgagttccaagctctaagaagatcgtttagtaagtacattgcaaccattacaggtgtcagagaaatagaaattccaagcggaagatctgcctttgtgtgtttaacctttgatgacttaactgaacaaactgagaatttgactccaatctgttatggttgtgaggctgtagaggtcagagtagaccatttggctaattactctgctgatttcgtgagtaaacagttatctatattgcgtaaagccactgacagtattcctatcatttttactgtgcgaaccatgaagcaaggtggcaactttcctgatgaagagttcaaaaccttgagagagctatacgatattgccttgaagaatggtgttgaattccttgacttagaactaactttacctactgatatccaatatgaggttattaacaaaaggggcaacaccaagatcattggttcccatcatgacttccaaggattatactcctgggacgacgctgaatgggaaaacagattcaatcaagcgttaactcttgatgtggatgttgtaaaatttgtgggtacggctgttaatttcgaagataatttgagactggaacactttagggatacacacaagaataagcctttaattgcagttaatatgacttctaaaggtagcatttctcgtgttttgaataatgttttaacacctgtgacatcagatttattgcctaactccgctgcccctggccaattgacagtagcacaaattaacaagatgtatacatctatgggaggtatcgagcctaaggaactgtttgttgttggaaagccaattggccactctagatcgccaattttacataacactggctatgaaattttaggtttacctcacaagttcgataaatttgaaactgaatccgcacaattggtgaaagaaaaacttttggacggaaacaagaactttggcggtgctgcagtcaggattcctctgaaattagatataatgcagtacatggatgaattgactgatgctgctaaagttattggtgctgtaaacacagttataccattgggtaacaagaagtttaagggtgataataccgactggttaggtatccgtaatgccttaattaacaatggcgttcccgaatatgttggtcataccgctggtttggttatcggtgcaggtggcacttctagagccgccctttacgccttgcacagtttaggttgcaaaaagatcttcataatcaacaggacaacttcgaaattgaagccattaatagagtcacttccatctgaattcaacattattggaatagagtccactaaatctatagaagagattaaggaacacgttggcgttgctgtcagctgtgtaccagccgacaaaccattagatgacgaacttttaagtaagctggagagattccttgtgaaaggtgcccatgctgcttttgtaccaaccttattggaagccgcatacaaaccaagcgttactcccgttatgacaatttcacaagacaaatatcaatggcacgttgtccctggatcacaaatgttagtacaccaaggtgtagctcagtttgaaaagtggacaggattcaagggccctttcaaggccatttttgatgccgttacgaaagagtag

SEQ ID NO: 14 - protein, 1588 aa, Artificial sequence
  Synthetic polypeptide
MVQLAKVPILGNDIIHVGYNIHDHLVETIIKHCPSSTYVICNDTNLSKVPYYQQLVLEFKASLPEGSRLLTYVVKPGETSKSRETKAQLEDYLLVEGCTRDTVMVAIGGGVIGDMIGFVASTFMRGVRVVQVPTSLLAMVDSSIGGKTAIDTPLGKNFIGAFWQPKFVLVDIKWLETLAKREFINGMAEVIKTACIWNADEFTRLESNASLFLNVVNGAKNVKVTNQLTNEIDEISNTDIEAMLDHTYKLVLESIKVKAEVVSSDERESSLRNLLNFGHSIGHAYEAILTPQALHGECVSIGMVKEAELSRYFGILSPTQVARLSKILVAYGLPVSPDEKWFKELTLHKKTPLDILLKKMSIDKKNEGSKKKVVILESIGKCYGDSAQFVSDEDLRFILTDETLVYPFKDIPADQQKVVIPPGSKSISNRALILAALGEGQCKIKNLLHSDDTKHMLTAVHELKGATISWEDNGETVVVEGHGGSTLSACADPLYLGNAGTASRFLTSLAALVNSTSSQKYIVLTGNARMQQRPIAPLVDSLRANGTKIEYLNNEGSLPIKVYTDSVFKGGRIELAATVSSQYVSSILMCAPYAEEPVTLALVGGKPISKLYVDMTIKMMEKFGINVETSTTEPYTYYIPKGHYINPSEYVIESDASSATYPLAFAAMTGTTVTVPNIGFESLQGDARFARDVLKPMGCKITQTATSTTVSGPPVGTLKPLKHVDMEPMTDAFLTACVVAAISHDSDPNSANTTTIEGIANQRVKECNRILAMATELAKFGVKTTELPDGIQVHGLNSIKDLKVPSDSSGPVGVCTYDDHRVAMSFSLLAGMVNSQNERDEVANPVRILERHCTGKTWPGWWDVLHSELGAKLDGAEPLECTSKKNSKKSVVIIGMRAAGKTTISKWCASALGYKLVDLDELFEQQHNNQSVKQFVVENGWEKFREEETRIFKEVIQNYGDDGYVFSTGGGIVESAESRKALKDFASSGGYVLHLHRDIEETIVFLQSDPSRPAYVEEIREVWNRREGWYKECSNFSFFAPHCSAEAEFQALRRSFSKYIATITGVREIEIPSGRSAFVCLTFDDLTEQTENLTPICYGCEAVEVRVDHLANYSADFVSKQLSILRKATDSIPIIFTVRTMKQGGNFPDEEFKTLRELYDIALKNGVEFLDLELTLPTDIQYEVINKRGNTKIIGSHHDFQGLYSWDDAEWENRFNQALTLDVDVVKFVGTAVNFEDNLRLEHFRDTHKNKPLIAVNMTSKGSISRVLNNVLTPVTSDLLPNSAAPGQLTVAQINKMYTSMGGIEPKELFVVGKPIGHSRSPILHNTGYEILGLPHKFDKFETESAQLVKEKLLDGNKNFGGAAVRIPLKLDIMQYMDELTDAAKVIGAVNTVIPLGNKKFKGDNTDWLGIRNALINNGVPEYVGHTAGLVIGAGGTSRAALYALHSLGCKKIFIINRTTSKLKPLIESLPSEFNIIGIESTKSIEEIKEHVGVAVSCVPADKPLDDELLSKLERFLVKGAHAAFVPTLLEAAYKPSVTPVMTISQDKYQWHVVPGSQMLVHQGVAQFEKWTGFKGPFKAIFDAVTKE

SEQ ID NO: 15 - DNA, 4767 bp, Artificial sequence
  Synthetic nucleic acid
atggtgcagttagccaaagtcccaattctaggaaatgatattatccacgttgggtataacattcatgaccatttggttgaaaccataattaaacattgtccttcttcgacatacgttatttgcaatgatacgaacttgagtaaagttccatactaccagcaattagtcctggaattcaaggcttctttgccagaaggctctcgtttacttacttatgttgttaaaccaggtgagacaagtaaaagtagagaaaccaaagcgcagctagaagattatcttttagtggaaggatgtactcgtgatacggttatggtagcgatcggtggtggtgttattggtgacatgattgggttcgttgcatctacatttatgagaggtgttcgtgttgtccaagtaccaacatccttattggcaatggtcgattcctccattggtggtaaaactgctattgacactcctctaggtaaaaactttattggtgcattttggcaaccaaaatttgtccttgtagatattaaatggctagaaacgttagccaagagagagtttatcaatgggatggcagaagttatcaagactgcttgtatttggaacgctgacgaatttactagattagaatcaaacgcttcgttgttcttaaatgttgttaatggggcaaaaaatgtcaaggttaccaatcaattgacaaacgagattgacgagatatcgaatacagatattgaagctatgttggatcatacatataagttagttcttgagagtattaaggtcaaagcggaagttgtctcttcggatgaacgtgaatccagtctaagaaaccttttgaacttcggacattctattggtcatgcttatgaagctatactaaccccacaagcattacatggtgaatgtgtgtccattggtatggttaaagaggcggaattatcccgttatttcggtattctctcccctacccaagttgcacgtctatccaagattttggttgcctacgggttgcctgtttcgcctgatgagaaatggtttaaagagctaaccttacataagaaaacaccattggatatcttattgaagaaaatgagtattgacaagaaaaacgagggttccaaaaagaaggtggtcattttagaaagtattggtaagtgctatggtgactccgctcaatttgttagcgatgaagacctgagatttattctaacagatgaaaccctcgtttaccccttcaaggacatccctgctgatcaacagaaagttgttatcccccctggttctaagtccatctccaatcgtgctttaattcttgctgccctcggtgaaggtcaatgtaaaatcaagaacttattacattctgatgatactaaacatatgttaaccgctgttcatgaattgaaaggtgctacgatatcatgggaagataatggtgagacggtagtggtggaaggacatggtggttccacattgtcagcttgtgctgaccccttatatctaggtaatgcaggtactgcatctagatttttgacttccttggctgccttggtcaattctacttcaagccaaaagtatatcgttttaactggtaacgcaagaatgcaacaaagaccaattgctcctttggtcgattctttgcgtgctaatggtactaaaattgagtacttgaataatgaaggttccctgccaatcaaagtttatactgattcggtattcaaaggtggtagaattgaattagctgctacagtttcttctcagtacgtatcctctatcttgatgtgtgccccatacgctgaagaacctgtaactttggctcttgttggtggtaagccaatctctaaattgtacgtcgatatgacaataaaaatgatggaaaaattcggtatcaatgttgaaacttctactacagaaccttacacttattatattccaaagggacattatattaacccatcagaatacgtcattgaaagtgatgcctcaagtgctacatacccattggccttcgccgcaatgactggtactaccgtaacggttccaaacattggttttgagtcgttacaaggtgatgccagatttgcaagagatgtcttgaaacctatgggttgtaaaataactcaaacggcaacttcaactactgtttcgggtcctcctgtaggtactttaaagccattaaaacatgttgatatggagccaatgactgatgcgttcttaactgcatgtgttgttgccgctatttcgcacgacagtgatccaaattctgcaaatacaaccaccattgaaggtattgcaaaccagcgtgtcaaagagtgtaacagaattttggccatggctacagagctcgccaaatttggcgtcaaaactacagaattaccagatggtattcaagtccatggtttaaactcgataaaagatttgaaggttccttccgactcttctggacctgtcggtgtatgcacatatgatgatcatcgtgtggccatgagtttctcgcttcttgcaggaatggtaaattctcaaaatgaacgtgacgaagttgctaatcctgtaagaatacttgaaagacattgtactggtaaaacctggcctggctggtgggatgtgttacattccgaactaggtgccaaattagatggtgcagaacctttagagtgcacatccaaaaagaactcaaagaaaagcgttgtcattattggcatgagagcagctggcaaaactactataagtaaatggtgcgcatccgctctgggttacaaattagttgacctagacgagctgtttgagcaacagcataacaatcaaagtgttaaacaatttgttgtggagaacggttgggagaagttccgtgaggaagaaacaagaattttcaaggaagttattcaaaattacggcgatgatggatatgttttctcaacaggtggcggtattgttgaaagcgctgagtctagaaaagccttaaaagattttgcctcatcaggtggatacgttttacacttacatagggatattgaggagacaattgtctttttacaaagtgatccttcaagacctgcctatgtggaagaaattcgtgaagtttggaacagaagggaggggtggtataaagaatgctcaaatttctctttctttgctcctcattgctccgcagaagctgagttccaagctctaagaagatcgtttagtaagtacattgcaaccattacaggtgtcagagaaatagaaattccaagcggaagatctgcctttgtgtgtttaacctttgatgacttaactgaacaaactgagaatttgactccaatctgttatggttgtgaggctgtagaggtcagagtagaccatttggctaattactctgctgatttcgtgagtaaacagttatctatattgcgtaaagccactgacagtattcctatcatttttactgtgcgaaccatgaagcaaggtggcaactttcctgatgaagagttcaaaaccttgagagagctatacgatattgccttgaagaatggtgttgaattccttgacttagaactaactttacctactgatatccaatatgaggttattaacaaaaggggcaacaccaagatcattggttcccatcatgacttccaaggattatactcctgggacgacgctgaatgggaaaacagattcaatcaagcgttaactcttgatgtggatgttgtaaaatttgtgggtacggctgttaatttcgaagataatttgagactggaacactttagggatacacacaagaataagcctttaattgcagttaatatgacttctaaaggtagcatttctcgtgttttgaataatgttttaacacctgtgacatcagatttattgcctaactccgctgcccctggccaattgacagtagcacaaattaacaagatgtatacatctatgggaggtatcgagcctaaggaactgtttgttgttggaaagccaattggccactctagatcgccaattttacataacactggctatgaaattttaggtttacctcacaagttcgataaatttgaaactgaatccgcacaattggtgaaagaaaaacttttggacggaaacaagaactttggcggtgctgcagtcacaattcctctgaaattagatataatgcagtacatggatgaattgactgatgctgctaaagttcatggtgctgtaaacacagttataccattgggtaacaagaagtttaagggtgataataccgactggttaggtatccgtaatgccttaattaacaatggcgttcccgaatatgttggtcataccgctggtttggttatcggtgcaggtggcacttctagagccgccctttacgccttgcacagtttaggttgcaaaaagatcttcataatcaacaggacaacttcgaaattgaagccattaatagagtcacttccatctgaattcaacattattggaatagagtccactaaatctatagaagagattaaggaacacgttggcgttgctgtcagctgtgtaccagccgacaaaccattagatgacgaacttttaagtaagctggagagattccttgtgaaaggtgcccatgctgcttttgtaccaaccttattggaagccgcatacaaaccaagcgttactcccgttatgacaatttcacaagacaaatatcaatggcacgttgtccctggatcacaaatgttagtacaccaaggtgtagctcagtttgaaaagtggacaggattcaagggccctttcaaggccatttttgatgccgttacgaaagagtag

SEQ ID NO: 16 - protein, 1588 aa, Artificial sequence
  Synthetic polypeptide
MVQLAKVPILGNDIIHVGYNIHDHLVETIIKHCPSSTYVICNDTNLSKVPYYQQLVLEFKASLPEGSRLLTYVVKPGETSKSRETKAQLEDYLLVEGCTRDTVMVAIGGGVIGDMIGFVASTFMRGVRVVQVPTSLLAMVDSSIGGKTAIDTPLGKNFIGAFWQPKFVLVDIKWLETLAKREFINGMAEVIKTACIWNADEFTRLESNASLFLNVVNGAKNVKVTNQLTNEIDEISNTDIEAMLDHTYKLVLESIKVKAEVVSSDERESSLRNLLNFGHSIGHAYEAILTPQALHGECVSIGMVKEAELSRYFGILSPTQVARLSKILVAYGLPVSPDEKWFKELTLHKKTPLDILLKKMSIDKKNEGSKKKVVILESIGKCYGDSAQFVSDEDLRFILTDETLVYPFKDIPADQQKVVIPPGSKSISNRALILAALGEGQCKIKNLLHSDDTKHMLTAVHELKGATISWEDNGETVVVEGHGGSTLSACADPLYLGNAGTASRFLTSLAALVNSTSSQKYIVLTGNARMQQRPIAPLVDSLRANGTKIEYLNNEGSLPIKVYTDSVFKGGRIELAATVSSQYVSSILMCAPYAEEPVTLALVGGKPISKLYVDMTIKMMEKFGINVETSTTEPYTYYIPKGHYINPSEYVIESDASSATYPLAFAAMTGTTVTVPNIGFESLQGDARFARDVLKPMGCKITQTATSTTVSGPPVGTLKPLKHVDMEPMTDAFLTACVVAAISHDSDPNSANTTTIEGIANQRVKECNRILAMATELAKFGVKTTELPDGIQVHGLNSIKDLKVPSDSSGPVGVCTYDDHRVAMSFSLLAGMVNSQNERDEVANPVRILERHCTGKTWPGWWDVLHSELGAKLDGAEPLECTSKKNSKKSVVIIGMRAAGKTTISKWCASALGYKLVDLDELFEQQHNNQSVKQFVVENGWEKFREEETRIFKEVIQNYGDDGYVFSTGGGIVESAESRKALKDFASSGGYVLHLHRDIEETIVFLQSDPSRPAYVEEIREVWNRREGWYKECSNFSFFAPHCSAEAEFQALRRSFSKYIATITGVREIEIPSGRSAFVCLTFDDLTEQTENLTPICYGCEAVEVRVDHLANYSADFVSKQLSILRKATDSIPIIFTVRTMKQGGNFPDEEFKTLRELYDIALKNGVEFLDLELTLPTDIQYEVINKRGNTKIIGSHHDFQGLYSWDDAEWENRFNQALTLDVDVVKFVGTAVNFEDNLRLEHFRDTHKNKPLIAVNMTSKGSISRVLNNVLTPVTSDLLPNSAAPGQLTVAQINKMYTSMGGIEPKELFVVGKPIGHSRSPILHNTGYEILGLPHKFDKFETESAQLVKEKLLDGNKNFGGAAVTIPLKLDIMQYMDELTDAAKVHGAVNTVIPLGNKKFKGDNTDWLGIRNALINNGVPEYVGHTAGLVIGAGGTSRAALYALHSLGCKKIFIINRTTSKLKPLIESLPSEFNIIGIESTKSIEEIKEHVGVAVSCVPADKPLDDELLSKLERFLVKGAHAAFVPTLLEAAYKPSVTPVMTISQDKYQWHVVPGSQMLVHQGVAQFEKWTGFKGPFKAIFDAVTKE

SEQ ID NO: 17 - DNA, 4767 bp, Artificial sequence
  Synthetic nucleic acid
atggtgcagttagccaaagtcccaattctaggaaatgatattatccacgttgggtataacattcatgaccatttggttgaaaccataattaaacattgtccttcttcgacatacgttatttgcaatgatacgaacttgagtaaagttccatactaccagcaattagtcctggaattcaaggcttctttgccagaaggctctcgtttacttacttatgttgttaaaccaggtgagacaagtaaaagtagagaaaccaaagcgcagctagaagattatcttttagtggaaggatgtactcgtgatacggttatggtagcgatcggtggtggtgttattggtgacatgattgggttcgttgcatctacatttatgagaggtgttcgtgttgtccaagtaccaacatccttattggcaatggtcgattcctccattggtggtaaaactgctattgacactcctctaggtaaaaactttattggtgcattttggcaaccaaaatttgtccttgtagatattaaatggctagaaacgttagccaagagagagtttatcaatgggatggcagaagttatcaagactgcttgtatttggaacgctgacgaatttactagattagaatcaaacgcttcgttgttcttaaatgttgttaatggggcaaaaaatgtcaaggttaccaatcaattgacaaacgagattgacgagatatcgaatacagatattgaagctatgttggatcatacatataagttagttcttgagagtattaaggtcaaagcggaagttgtctcttcggatgaacgtgaatccagtctaagaaaccttttgaacttcggacattctattggtcatgcttatgaagctatactaaccccacaagcattacatggtgaatgtgtgtccattggtatggttaaagaggcggaattatcccgttatttcggtattctctcccctacccaagttgcacgtctatccaagattttggttgcctacgggttgcctgtttcgcctgatgagaaatggtttaaagagctaaccttacataagaaaacaccattggatatcttattgaagaaaatgagtattgacaagaaaaacgagggttccaaaaagaaggtggtcattttagaaagtattggtaagtgctatggtgactccgctcaatttgttagcgatgaagacctgagatttattctaacagatgaaaccctcgtttaccccttcaaggacatccctgctgatcaacagaaagttgttatcccccctggttctaagtccatctccaatcgtgctttaattcttgctgccctcggtgaaggtcaatgtaaaatcaagaacttattacattctgatgatactaaacatatgttaaccgctgttcatgaattgaaaggtgctacgatatcatgggaagataatggtgagacggtagtggtggaaggacatggtggttccacattgtcagcttgtgctgaccccttatatctaggtaatgcaggtactgcatctagatttttgacttccttggctgccttggtcaattctacttcaagccaaaagtatatcgttttaactggtaacgcaagaatgcaacaaagaccaattgctcctttggtcgattctttgcgtgctaatggtactaaaattgagtacttgaataatgaaggttccctgccaatcaaagtttatactgattcggtattcaaaggtggtagaattgaattagctgctacagtttcttctcagtacgtatcctctatcttgatgtgtgccccatacgctgaagaacctgtaactttggctcttgttggtggtaagccaatctctaaattgtacgtcgatatgacaataaaaatgatggaaaaattcggtatcaatgttgaaacttctactacagaaccttacacttattatattccaaagggacattatattaacccatcagaatacgtcattgaaagtgatgcctcaagtgctacatacccattggccttcgccgcaatgactggtactaccgtaacggttccaaacattggttttgagtcgttacaaggtgatgccagatttgcaagagatgtcttgaaacctatgggttgtaaaataactcaaacggcaacttcaactactgtttcgggtcctcctgtaggtactttaaagccattaaaacatgttgatatggagccaatgactgatgcgttcttaactgcatgtgttgttgccgctatttcgcacgacagtgatccaaattctgcaaatacaaccaccattgaaggtattgcaaaccagcgtgtcaaagagtgtaacagaattttggccatggctacagagctcgccaaatttggcgtcaaaactacagaattaccagatggtattcaagtccatggtttaaactcgataaaagatttgaaggttccttccgactcttctggacctgtcggtgtatgcacatatgatgatcatcgtgtggccatgagtttctcgcttcttgcaggaatggtaaattctcaaaatgaacgtgacgaagttgctaatcctgtaagaatacttgaaagacattgtactggtaaaacctggcctggctggtgggatgtgttacattccgaactaggtgccaaattagatggtgcagaacctttagagtgcacatccaaaaagaactcaaagaaaagcgttgtcattattggcatgagagcagctggcaaaactactataagtaaatggtgcgcatccgctctgggttacaaattagttgacctagacgagctgtttgagcaacagcataacaatcaaagtgttaaacaatttgttgtggagaacggttgggagaagttccgtgaggaagaaacaagaattttcaaggaagttattcaaaattacggcgatgatggatatgttttctcaacaggtggcggtattgttgaaagcgctgagtctagaaaagccttaaaagattttgcctcatcaggtggatacgttttacacttacatagggatattgaggagacaattgtctttttacaaagtgatccttcaagacctgcctatgtggaagaaattcgtgaagtttggaacagaagggaggggtggtataaagaatgctcaaatttctctttctttgctcctcattgctccgcagaagctgagttccaagctctaagaagatcgtttagtaagtacattgcaaccattacaggtgtcagagaaatagaaattccaagcggaagatctgcctttgtgtgtttaacctttgatgacttaactgaacaaactgagaatttgactccaatctgttatggttgtgaggctgtagaggtcagagtagaccatttggctaattactctgctgatttcgtgagtaaacagttatctatattgcgtaaagccactgacagtattcctatcatttttactgtgcgaaccatgaagcaaggtggcaactttcctgatgaagagttcaaaaccttgagagagctatacgatattgccttgaagaatggtgttgaattccttgacttagaactaactttacctactgatatccaatatgaggttattaacaaaaggggcaacaccaagatcattggttcccatcatgacttccaaggattatactcctgggacgacgctgaatgggaaaacagattcaatcaagcgttaactcttgatgtggatgttgtaaaatttgtgggtacggctgttaatttcgaagataatttgagactggaacactttagggatacacacaagaataagcctttaattgcagttaatatgacttctaaaggtagcatttctcgtgttttgaataatgttttaacacctgtgacatcagatttattgcctaactccgctgcccctggccaattgacagtagcacaaattaacaagatgtatacatctatgggaggtatcgagcctaaggaactgtttgttgttggaaagccaattggccactctagatcgccaattttacataacactggctatgaaattttaggtttacctcacaagttcgataaatttgaaactgaatccgcacaattggtgaaagaaaaacttttggacggaaacaagaactttggcggtgctgcagtcacaattcctctgaaattagatataatgcagtacatggatgaattgactgatgctgctaaagttattggtgctgtaaacacagttataccattgggtaacaagaagtttaagggtgataataccgactggttaggtatccgtaatgccttaattaacaatggcgttcccgaatatgttggtcataccgctggtttggttatcggtgcaggtggcacttctagagccgccctttacgccttgcacagtttaggttgcaaaaagatcttcataatcaacaggacaacttcgaaattgaagccattaatagagtcacttccatctgaattcaacattattggaatagagtccactaaatctatagaagagattaaggaacacgttggcgttgctgtcagctgtgtaccagccgacaaaccattagatgacgaacttttaagtaagctggagagattccttgtgaaaggtgcccatgctgcttttgtaccaaccttattggaagccgcatacaaaccaagcgttactcccgttatgacaatttcacaagacaaatatcaatggcacgttgtccctggatcacaaatgttagtacaccaaggtgtagctcagtttgaaaaggttacaggattcaagggccctttcaaggccatttttgatgccgttacgaaagagtag

SEQ ID NO: 18 - protein, 1588 aa, Artificial sequence
  Synthetic polypeptide
MVQLAKVPILGNDIIHVGYNIHDHLVETIIKHCPSSTYVICNDTNLSKVPYYQQLVLEFKASLPEGSRLLTYVVKPGETSKSRETKAQLEDYLLVEGCTRDTVMVAIGGGVIGDMIGFVASTFMRGVRVVQVPTSLLAMVDSSIGGKTAIDTPLGKNFIGAFWQPKFVLVDIKWLETLAKREFINGMAEVIKTACIWNADEFTRLESNASLFLNVVNGAKNVKVTNQLTNEIDEISNTDIEAMLDHTYKLVLESIKVKAEVVSSDERESSLRNLLNFGHSIGHAYEAILTPQALHGECVSIGMVKEAELSRYFGILSPTQVARLSKILVAYGLPVSPDEKWFKELTLHKKTPLDILLKKMSIDKKNEGSKKKVVILESIGKCYGDSAQFVSDEDLRFILTDETLVYPFKDIPADQQKVVIPPGSKSISNRALILAALGEGQCKIKNLLHSDDTKHMLTAVHELKGATISWEDNGETVVVEGHGGSTLSACADPLYLGNAGTASRFLTSLAALVNSTSSQKYIVLTGNARMQQRPIAPLVDSLRANGTKIEYLNNEGSLPIKVYTDSVFKGGRIELAATVSSQYVSSILMCAPYAEEPVTLALVGGKPISKLYVDMTIKMMEKFGINVETSTTEPYTYYIPKGHYINPSEYVIESDASSATYPLAFAAMTGTTVTVPNIGFESLQGDARFARDVLKPMGCKITQTATSTTVSGPPVGTLKPLKHVDMEPMTDAFLTACVVAAISHDSDPNSANTTTIEGIANQRVKECNRILAMATELAKFGVKTTELPDGIQVHGLNSIKDLKVPSDSSGPVGVCTYDDHRVAMSFSLLAGMVNSQNERDEVANPVRILERHCTGKTWPGWWDVLHSELGAKLDGAEPLECTSKKNSKKSVVIIGMRAAGKTTISKWCASALGYKLVDLDELFEQQHNNQSVKQFVVENGWEKFREEETRIFKEVIQNYGDDGYVFSTGGGIVESAESRKALKDFASSGGYVLHLHRDIEETIVFLQSDPSRPAYVEEIREVWNRREGWYKECSNFSFFAPHCSAEAEFQALRRSFSKYIATITGVREIEIPSGRSAFVCLTFDDLTEQTENLTPICYGCEAVEVRVDHLANYSADFVSKQLSILRKATDSIPIIFTVRTMKQGGNFPDEEFKTLRELYDIALKNGVEFLDLELTLPTDIQYEVINKRGNTKIIGSHHDFQGLYSWDDAEWENRFNQALTLDVDVVKFVGTAVNFEDNLRLEHFRDTHKNKPLIAVNMTSKGSISRVLNNVLTPVTSDLLPNSAAPGQLTVAQINKMYTSMGGIEPKELFVVGKPIGHSRSPILHNTGYEILGLPHKFDKFETESAQLVKEKLLDGNKNFGGAAVTIPLKLDIMQYMDELTDAAKVIGAVNTVIPLGNKKFKGDNTDWLGIRNALINNGVPEYVGHTAGLVIGAGGTSRAALYALHSLGCKKIFIINRTTSKLKPLIESLPSEFNIIGIESTKSIEEIKEHVGVAVSCVPADKPLDDELLSKLERFLVKGAHAAFVPTLLEAAYKPSVTPVMTISQDKYQWHVVPGSQMLVHQGVAQFEKVTGFKGPFKAIFDAVTKE

SEQ ID NO: 19 - DNA, 4767 bp, Artificial sequence
  Synthetic nucleic acid
atggtgcagttagccaaagtcccaattctaggaaatgatattatccacgttgggtataacattcatgaccatttggttgaaaccataattaaacattgtccttcttcgacatacgttatttgcaatgatacgaacttgagtaaagttccatactaccagcaattagtcctggaattcaaggcttctttgccagaaggctctcgtttacttacttatgttgttaaaccaggtgagacaagtaaaagtagagaaaccaaagcgcagctagaagattatcttttagtggaaggatgtactcgtgatacggttatggtagcgatcggtggtggtgttattggtgacatgattgggttcgttgcatctacatttatgagaggtgttcgtgttgtccaagtaccaacatccttattggcaatggtcgattcctccattggtggtaaaactgctattgacactcctctaggtaaaaactttattggtgcattttggcaaccaaaatttgtccttgtagatattaaatggctagaaacgttagccaagagagagtttatcaatgggatggcagaagttatcaagactgcttgtatttggaacgctgacgaatttactagattagaatcaaacgcttcgttgttcttaaatgttgttaatggggcaaaaaatgtcaaggttaccaatcaattgacaaacgagattgacgagatatcgaatacagatattgaagctatgttggatcatacatataagttagttcttgagagtattaaggtcaaagcggaagttgtctcttcggatgaacgtgaatccagtctaagaaaccttttgaacttcggacattctattggtcatgcttatgaagctatactaaccccacaagcattacatggtgaatgtgtgtccattggtatggttaaagaggcggaattatcccgttatttcggtattctctcccctacccaagttgcacgtctatccaagattttggttgcctacgggttgcctgtttcgcctgatgagaaatggtttaaagagctaaccttacataagaaaacaccattggatatcttattgaagaaaatgagtattgacaagaaaaacgagggttccaaaaagaaggtggtcattttagaaagtattggtaagtgctatggtgactccgctcaatttgttagcgatgaagacctgagatttattctaacagatgaaaccctcgtttaccccttcaaggacatccctgctgatcaacagaaagttgttatcccccctggttctaagtccatctccaatcgtgctttaattcttgctgccctcggtgaaggtcaatgtaaaatcaagaacttattacattctgatgatactaaacatatgttaaccgctgttcatgaattgaaaggtgctacgatatcatgggaagataatggtgagacggtagtggtggaaggacatggtggttccacattgtcagcttgtgctgaccccttatatctaggtaatgcaggtactgcatctagatttttgacttccttggctgccttggtcaattctacttcaagccaaaagtatatcgttttaactggtaacgcaagaatgcaacaaagaccaattgctcctttggtcgattctttgcgtgctaatggtactaaaattgagtacttgaataatgaaggttccctgccaatcaaagtttatactgattcggtattcaaaggtggtagaattgaattagctgctacagtttcttctcagtacgtatcctctatcttgatgtgtgccccatacgctgaagaacctgtaactttggctcttgttggtggtaagccaatctctaaattgtacgtcgatatgacaataaaaatgatggaaaaattcggtatcaatgttgaaacttctactacagaaccttacacttattatattccaaagggacattatattaacccatcagaatacgtcattgaaagtgatgcctcaagtgctacatacccattggccttcgccgcaatgactggtactaccgtaacggttccaaacattggttttgagtcgttacaaggtgatgccagatttgcaagagatgtcttgaaacctatgggttgtaaaataactcaaacggcaacttcaactactgtttcgggtcctcctgtaggtactttaaagccattaaaacatgttgatatggagccaatgactgatgcgttcttaactgcatgtgttgttgccgctatttcgcacgacagtgatccaaattctgcaaatacaaccaccattgaaggtattgcaaaccagcgtgtcaaagagtgtaacagaattttggccatggctacagagctcgccaaatttggcgtcaaaactacagaattaccagatggtattcaagtccatggtttaaactcgataaaagatttgaaggttccttccgactcttctggacctgtcggtgtatgcacatatgatgatcatcgtgtggccatgagtttctcgcttcttgcaggaatggtaaattctcaaaatgaacgtgacgaagttgctaatcctgtaagaatacttgaaagacattgtactggtaaaacctggcctggctggtgggatgtgttacattccgaactaggtgccaaattagatggtgcagaacctttagagtgcacatccaaaaagaactcaaagaaaagcgttgtcattattggcatgagagcagctggcaaaactactataagtaaatggtgcgcatccgctctgggttacaaattagttgacctagacgagctgtttgagcaacagcataacaatcaaagtgttaaacaatttgttgtggagaacggttgggagaagttccgtgaggaagaaacaagaattttcaaggaagttattcaaaattacggcgatgatggatatgttttctcaacaggtggcggtattgttgaaagcgctgagtctagaaaagccttaaaagattttgcctcatcaggtggatacgttttacacttacatagggatattgaggagacaattgtctttttacaaagtgatccttcaagacctgcctatgtggaagaaattcgtgaagtttggaacagaagggaggggtggtataaagaatgctcaaatttctctttctttgctcctcattgctccgcagaagctgagttccaagctctaagaagatcgtttagtaagtacattgcaaccattacaggtgtcagagaaatagaaattccaagcggaagatctgcctttgtgtgtttaacctttgatgacttaactgaacaaactgagaatttgactccaatctgttatggttgtgaggctgtagaggtcagagtagaccatttggctaattactctgctgatttcgtgagtaaacagttatctatattgcgtaaagccactgacagtattcctatcatttttactgtgcgaaccatgaagcaaggtggcaactttcctgatgaagagttcaaaaccttgagagagctatacgatattgccttgaagaatggtgttgaattccttgacttagaactaactttacctactgatatccaatatgaggttattaacaaaaggggcaacaccaagatcattggttcccatcatgacttccaaggattatactcctgggacgacgctgaatgggaaaacagattcaatcaagcgttaactcttgatgtggatgttgtaaaatttgtgggtacggctgttaatttcgaagataatttgagactggaacactttagggatacacacaagaataagcctttaattgcagttaatatgacttctaaaggtagcatttctcgtgttttgaataatgttttaacacctgtgacatcagatttattgcctaactccgctgcccctggccaattgacagtagcacaaattaacaagatgtatacatctatgggaggtatcgagcctaaggaactgtttgttgttggaaagccaattggccactctagatcgccaattttacataacactggctatgaaattttaggtttacctcacaagttcgataaatttgaaactgaatccgcacaattggtgaaagaaaaacttttggacggaaacaagaactttggcggtgctgcagtcacaattcctctgaaattagatataatgcagtacatggatgaattgactgatgctgctaaagttattggtgctgtaaacaaagttataccattgggtaacaagaagtttaagggtgataataccgactggttaggtatccgtaatgccttaattaacaatggcgttcccgaatatgttggtcataccgctggtttggttatcggtgcaggtggcacttctagagccgccctttacgccttgcacagtttaggttgcaaaaagatcttcataatcaacaggacaacttcgaaattgaagccattaatagagtcacttccatctgaattcaacattattggaatagagtccactaaatctatagaagagattaaggaacacgttggcgttgctgtcagctgtgtaccagccgacaaaccattagatgacgaacttttaagtaagctggagagattccttgtgaaaggtgcccatgctgcttttgtaccaaccttattggaagccgcatacaaaccaagcgttactcccgttatgacaatttcacaagacaaatatcaatggcacgttgtccctggatcacaaatgttagtacaccaaggtgtagctcagtttgaaaagtggacaggattcaagggccctttcaaggccatttttgatgccgttacgaaagagtag

SEQ ID NO: 20 - protein, 1588 aa, Artificial sequence
  Synthetic polypeptide
MVQLAKVPILGNDIIHVGYNIHDHLVETIIKHCPSSTYVICNDTNLSKVPYYQQLVLEFKASLPEGSRLLTYVVKPGETSKSRETKAQLEDYLLVEGCTRDTVMVAIGGGVIGDMIGFVASTFMRGVRVVQVPTSLLAMVDSSIGGKTAIDTPLGKNFIGAFWQPKFVLVDIKWLETLAKREFINGMAEVIKTACIWNADEFTRLESNASLFLNVVNGAKNVKVTNQLTNEIDEISNTDIEAMLDHTYKLVLESIKVKAEVVSSDERESSLRNLLNFGHSIGHAYEAILTPQALHGECVSIGMVKEAELSRYFGILSPTQVARLSKILVAYGLPVSPDEKWFKELTLHKKTPLDILLKKMSIDKKNEGSKKKVVILESIGKCYGDSAQFVSDEDLRFILTDETLVYPFKDIPADQQKVVIPPGSKSISNRALILAALGEGQCKIKNLLHSDDTKHMLTAVHELKGATISWEDNGETVVVEGHGGSTLSACADPLYLGNAGTASRFLTSLAALVNSTSSQKYIVLTGNARMQQRPIAPLVDSLRANGTKIEYLNNEGSLPIKVYTDSVFKGGRIELAATVSSQYVSSILMCAPYAEEPVTLALVGGKPISKLYVDMTIKMMEKFGINVETSTTEPYTYYIPKGHYINPSEYVIESDASSATYPLAFAAMTGTTVTVPNIGFESLQGDARFARDVLKPMGCKITQTATSTTVSGPPVGTLKPLKHVDMEPMTDAFLTACVVAAISHDSDPNSANTTTIEGIANQRVKECNRILAMATELAKFGVKTTELPDGIQVHGLNSIKDLKVPSDSSGPVGVCTYDDHRVAMSFSLLAGMVNSQNERDEVANPVRILERHCTGKTWPGWWDVLHSELGAKLDGAEPLECTSKKNSKKSVVIIGMRAAGKTTISKWCASALGYKLVDLDELFEQQHNNQSVKQFVVENGWEKFREEETRIFKEVIQNYGDDGYVFSTGGGIVESAESRKALKDFASSGGYVLHLHRDIEETIVFLQSDPSRPAYVEEIREVWNRREGWYKECSNFSFFAPHCSAEAEFQALRRSFSKYIATITGVREIEIPSGRSAFVCLTFDDLTEQTENLTPICYGCEAVEVRVDHLANYSADFVSKQLSILRKATDSIPIIFTVRTMKQGGNFPDEEFKTLRELYDIALKNGVEFLDLELTLPTDIQYEVINKRGNTKIIGSHHDFQGLYSWDDAEWENRFNQALTLDVDVVKFVGTAVNFEDNLRLEHFRDTHKNKPLIAVNMTSKGSISRVLNNVLTPVTSDLLPNSAAPGQLTVAQINKMYTSMGGIEPKELFVVGKPIGHSRSPILHNTGYEILGLPHKFDKFETESAQLVKEKLLDGNKNFGGAAVTIPLKLDIMQYMDELTDAAKVIGAVNKVIPLGNKKFKGDNTDWLGIRNALINNGVPEYVGHTAGLVIGAGGTSRAALYALHSLGCKKIFIINRTTSKLKPLIESLPSEFNIIGIESTKSIEEIKEHVGVAVSCVPADKPLDDELLSKLERFLVKGAHAAFVPTLLEAAYKPSVTPVMTISQDKYQWHVVPGSQMLVHQGVAQFEKWTGFKGPFKAIFDAVTKE

SEQ ID NO: 21 - DNA, 4767 bp, Artificial sequence
  Synthetic nucleic acid
atggtgcagttagccaaagtcccaattctaggaaatgatattatccacgttgggtataacattcatgaccatttggttgaaaccataattaaacattgtccttcttcgacatacgttatttgcaatgatacgaacttgagtaaagttccatactaccagcaattagtcctggaattcaaggcttctttgccagaaggctctcgtttacttacttatgttgttaaaccaggtgagacaagtaaaagtagagaaaccaaagcgcagctagaagattatcttttagtggaaggatgtactcgtgatacggttatggtagcgatcggtggtggtgttattggtgacatgattgggttcgttgcatctacatttatgagaggtgttcgtgttgtccaagtaccaacatccttattggcaatggtcgattcctccattggtggtaaaactgctattgacactcctctaggtaaaaactttattggtgcattttggcaaccaaaatttgtccttgtagatattaaatggctagaaacgttagccaagagagagtttatcaatgggatggcagaagttatcaagactgcttgtatttggaacgctgacgaatttactagattagaatcaaacgcttcgttgttcttaaatgttgttaatggggcaaaaaatgtcaaggttaccaatcaattgacaaacgagattgacgagatatcgaatacagatattgaagctatgttggatcatacatataagttagttcttgagagtattaaggtcaaagcggaagttgtctcttcggatgaacgtgaatccagtctaagaaaccttttgaacttcggacattctattggtcatgcttatgaagctatactaaccccacaagcattacatggtgaatgtgtgtccattggtatggttaaagaggcggaattatcccgttatttcggtattctctcccctacccaagttgcacgtctatccaagattttggttgcctacgggttgcctgtttcgcctgatgagaaatggtttaaagagctaaccttacataagaaaacaccattggatatcttattgaagaaaatgagtattgacaagaaaaacgagggttccaaaaagaaggtggtcattttagaaagtattggtaagtgctatggtgactccgctcaatttgttagcgatgaagacctgagatttattctaacagatgaaaccctcgtttaccccttcaaggacatccctgctgatcaacagaaagttgttatcccccctggttctaagtccatctccaatcgtgctttaattcttgctgccctcggtgaaggtcaatgtaaaatcaagaacttattacattctgatgatactaaacatatgttaaccgctgttcatgaattgaaaggtgctacgatatcatgggaagataatggtgagacggtagtggtggaaggacatggtggttccacattgtcagcttgtgctgaccccttatatctaggtaatgcaggtactgcatctagatttttgacttccttggctgccttggtcaattctacttcaagccaaaagtatatcgttttaactggtaacgcaagaatgcaacaaagaccaattgctcctttggtcgattctttgcgtgctaatggtactaaaattgagtacttgaataatgaaggttccctgccaatcaaagtttatactgattcggtattcaaaggtggtagaattgaattagctgctacagtttcttctcagtacgtatcctctatcttgatgtgtgccccatacgctgaagaacctgtaactttggctcttgttggtggtaagccaatctctaaattgtacgtcgatatgacaataaaaatgatggaaaaattcggtatcaatgttgaaacttctactacagaaccttacacttattatattccaaagggacattatattaacccatcagaatacgtcattgaaagtgatgcctcaagtgctacatacccattggccttcgccgcaatgactggtactaccgtaacggttccaaacattggttttgagtcgttacaaggtgatgccagatttgcaagagatgtcttgaaacctatgggttgtaaaataactcaaacggcaacttcaactactgtttcgggtcctcctgtaggtactttaaagccattaaaacatgttgatatggagccaatgactgatgcgttcttaactgcatgtgttgttgccgctatttcgcacgacagtgatccaaattctgcaaatacaaccaccattgaaggtattgcaaaccagcgtgtcaaagagtgtaacagaattttggccatggctacagagctcgccaaatttggcgtcaaaactacagaattaccagatggtattcaagtccatggtttaaactcgataaaagatttgaaggttccttccgactcttctggacctgtcggtgtatgcacatatgatgatcatcgtgtggccatgagtttctcgcttcttgcaggaatggtaaattctcaaaatgaacgtgacgaagttgctaatcctgtaagaatacttgaaagacattgtactggtaaaacctggcctggctggtgggatgtgttacattccgaactaggtgccaaattagatggtgcagaacctttagagtgcacatccaaaaagaactcaaagaaaagcgttgtcattattggcatgagagcagctggcaaaactactataagtaaatggtgcgcatccgctctgggttacaaattagttgacctagacgagctgtttgagcaacagcataacaatcaaagtgttaaacaatttgttgtggagaacggttgggagaagttccgtgaggaagaaacaagaattttcaaggaagttattcaaaattacggcgatgatggatatgttttctcaacaggtggcggtattgttgaaagcgctgagtctagaaaagccttaaaagattttgcctcatcaggtggatacgttttacacttacatagggatattgaggagacaattgtctttttacaaagtgatccttcaagacctgcctatgtggaagaaattcgtgaagtttggaacagaagggaggggtggtataaagaatgctcaaatttctctttctttgctcctcattgctccgcagaagctgagttccaagctctaagaagatcgtttagtaagtacattgcaaccattacaggtgtcagagaaatagaaattccaagcggaagatctgcctttgtgtgtttaacctttgatgacttaactgaacaaactgagaatttgactccaatctgttatggttgtgaggctgtagaggtcagagtagaccatttggctaattactctgctgatttcgtgagtaaacagttatctatattgcgtaaagccactgacagtattcctatcatttttactgtgcgaaccatgaagcaaggtggcaactttcctgatgaagagttcaaaaccttgagagagctatacgatattgccttgaagaatggtgttgaattccttgacttagaactaactttacctactgatatccaatatgaggttattaacaaaaggggcaacaccaagatcattggttcccatcatgacttccaaggattatactcctgggacgacgctgaatgggaaaacagattcaatcaagcgttaactcttgatgtggatgttgtaaaatttgtgggtacggctgttaatttcgaagataatttgagactggaacactttagggatacacacaagaataagcctttaattgcagttaatatgacttctaaaggtagcatttctcgtgttttgaataatgttttaacacctgtgacatcagatttattgcctaactccgctgcccctggccaattgacagtagcacaaattaacaagatgtatacatctatgggaggtatcgagcctaaggaactgtttgttgttggaaagccaattggccactctagatcgccaattttacataacactggctatgaaattttaggtttacctcacaagttcgataaatttgaaactgaatccgcacaattggtgaaagaaaaacttttggacggaaacaagaactttggcggtgctgcagtcacaattcctctgttattagatataatgcagtacatggatgaattgactgatgctgctaaagttattggtgctgtaaacacagttataccattgggtaacaagaagtttaagggtgataataccgactggttaggtatccgtaatgccttaattaacaatggcgttcccgaatatgttggtcataccgctggtttggttatcggtgcaggtggcacttctagagccgccctttacgccttgcacagtttaggttgcaaaaagatcttcataatcaacaggacaacttcgaaattgaagccattaatagagtcacttccatctgaattcaacattattggaatagagtccactaaatctatagaagagattaaggaacacgttggcgttgctgtcagctgtgtaccagccgacaaaccattagatgacgaacttttaagtaagctggagagattccttgtgaaaggtgcccatgctgcttttgtaccaaccttattggaagccgcatacaaaccaagcgttactcccgttatgacaatttcacaagacaaatatcaatggcacgttgtccctggatcacaaatgttagtacaccaaggtgtagctcagtttgaaaagtggacaggattcaagggccctttcaaggccatttttgatgccgttacgaaagagtag

SEQ ID NO: 22 - protein, 1588 aa, Artificial sequence
  Synthetic polypeptide
MVQLAKVPILGNDIIHVGYNIHDHLVETIIKHCPSSTYVICNDTNLSKVPYYQQLVLEFKASLPEGSRLLTYVVKPGETSKSRETKAQLEDYLLVEGCTRDTVMVAIGGGVIGDMIGFVASTFMRGVRVVQVPTSLLAMVDSSIGGKTAIDTPLGKNFIGAFWQPKFVLVDIKWLETLAKREFINGMAEVIKTACIWNADEFTRLESNASLFLNVVNGAKNVKVTNQLTNEIDEISNTDIEAMLDHTYKLVLESIKVKAEVVSSDERESSLRNLLNFGHSIGHAYEAILTPQALHGECVSIGMVKEAELSRYFGILSPTQVARLSKILVAYGLPVSPDEKWFKELTLHKKTPLDILLKKMSIDKKNEGSKKKVVILESIGKCYGDSAQFVSDEDLRFILTDETLVYPFKDIPADQQKVVIPPGSKSISNRALILAALGEGQCKIKNLLHSDDTKHMLTAVHELKGATISWEDNGETVVVEGHGGSTLSACADPLYLGNAGTASRFLTSLAALVNSTSSQKYIVLTGNARMQQRPIAPLVDSLRANGTKIEYLNNEGSLPIKVYTDSVFKGGRIELAATVSSQYVSSILMCAPYAEEPVTLALVGGKPISKLYVDMTIKMMEKFGINVETSTTEPYTYYIPKGHYINPSEYVIESDASSATYPLAFAAMTGTTVTVPNIGFESLQGDARFARDVLKPMGCKITQTATSTTVSGPPVGTLKPLKHVDMEPMTDAFLTACVVAAISHDSDPNSANTTTIEGIANQRVKECNRILAMATELAKFGVKTTELPDGIQVHGLNSIKDLKVPSDSSGPVGVCTYDDHRVAMSFSLLAGMVNSQNERDEVANPVRILERHCTGKTWPGWWDVLHSELGAKLDGAEPLECTSKKNSKKSVVIIGMRAAGKTTISKWCASALGYKLVDLDELFEQQHNNQSVKQFVVENGWEKFREEETRIFKEVIQNYGDDGYVFSTGGGIVESAESRKALKDFASSGGYVLHLHRDIEETIVFLQSDPSRPAYVEEIREVWNRREGWYKECSNFSFFAPHCSAEAEFQALRRSFSKYIATITGVREIEIPSGRSAFVCLTFDDLTEQTENLTPICYGCEAVEVRVDHLANYSADFVSKQLSILRKATDSIPIIFTVRTMKQGGNFPDEEFKTLRELYDIALKNGVEFLDLELTLPTDIQYEVINKRGNTKIIGSHHDFQGLYSWDDAEWENRFNQALTLDVDVVKFVGTAVNFEDNLRLEHFRDTHKNKPLIAVNMTSKGSISRVLNNVLTPVTSDLLPNSAAPGQLTVAQINKMYTSMGGIEPKELFVVGKPIGHSRSPILHNTGYEILGLPHKFDKFETESAQLVKEKLLDGNKNFGGAAVTIPLLLDIMQYMDELTDAAKVIGAVNTVIPLGNKKFKGDNTDWLGIRNALINNGVPEYVGHTAGLVIGAGGTSRAALYALHSLGCKKIFIINRTTSKLKPLIESLPSEFNIIGIESTKSIEEIKEHVGVAVSCVPADKPLDDELLSKLERFLVKGAHAAFVPTLLEAAYKPSVTPVMTISQDKYQWHVVPGSQMLVHQGVAQFEKWTGFKGPFKAIFDAVTKE

SEQ ID NO: 23 - DNA, 4767 bp, Artificial sequence
  Synthetic nucleic acid
atggtgcagttagccaaagtcccaattctaggaaatgatattatccacgttgggtataacattcatgaccatttggttgaaaccataattaaacattgtccttcttcgacatacgttatttgcaatgatacgaacttgagtaaagttccatactaccagcaattagtcctggaattcaaggcttctttgccagaaggctctcgtttacttacttatgttgttaaaccaggtgagacaagtaaaagtagagaaaccaaagcgcagctagaagattatcttttagtggaaggatgtactcgtgatacggttatggtagcgatcggtggtggtgttattggtgacatgattgggttcgttgcatctacatttatgagaggtgttcgtgttgtccaagtaccaacatccttattggcaatggtcgattcctccattggtggtaaaactgctattgacactcctctaggtaaaaactttattggtgcattttggcaaccaaaatttgtccttgtagatattaaatggctagaaacgttagccaagagagagtttatcaatgggatggcagaagttatcaagactgcttgtatttggaacgctgacgaatttactagattagaatcaaacgcttcgttgttcttaaatgttgttaatggggcaaaaaatgtcaaggttaccaatcaattgacaaacgagattgacgagatatcgaatacagatattgaagctatgttggatcatacatataagttagttcttgagagtattaaggtcaaagcggaagttgtctcttcggatgaacgtgaatccagtctaagaaaccttttgaacttcggacattctattggtcatgcttatgaagctatactaaccccacaagcattacatggtgaatgtgtgtccattggtatggttaaagaggcggaattatcccgttatttcggtattctctcccctacccaagttgcacgtctatccaagattttggttgcctacgggttgcctgtttcgcctgatgagaaatggtttaaagagctaaccttacataagaaaacaccattggatatcttattgaagaaaatgagtattgacaagaaaaacgagggttccaaaaagaaggtggtcattttagaaagtattggtaagtgctatggtgactccgctcaatttgttagcgatgaagacctgagatttattctaacagatgaaaccctcgtttaccccttcaaggacatccctgctgatcaacagaaagttgttatcccccctggttctaagtccatctccaatcgtgctttaattcttgctgccctcggtgaaggtcaatgtaaaatcaagaacttattacattctgatgatactaaacatatgttaaccgctgttcatgaattgaaaggtgctacgatatcatgggaagataatggtgagacggtagtggtggaaggacatggtggttccacattgtcagcttgtgctgaccccttatatctaggtaatgcaggtactgcatctagatttttgacttccttggctgccttggtcaattctacttcaagccaaaagtatatcgttttaactggtaacgcaagaatgcaacaaagaccaattgctcctttggtcgattctttgcgtgctaatggtactaaaattgagtacttgaataatgaaggttccctgccaatcaaagtttatactgattcggtattcaaaggtggtagaattgaattagctgctacagtttcttctcagtacgtatcctctatcttgatgtgtgccccatacgctgaagaacctgtaactttggctcttgttggtggtaagccaatctctaaattgtacgtcgatatgacaataaaaatgatggaaaaattcggtatcaatgttgaaacttctactacagaaccttacacttattatattccaaagggacattatattaacccatcagaatacgtcattgaaagtgatgcctcaagtgctacatacccattggccttcgccgcaatgactggtactaccgtaacggttccaaacattggttttgagtcgttacaaggtgatgccagatttgcaagagatgtcttgaaacctatgggttgtaaaataactcaaacggcaacttcaactactgtttcgggtcctcctgtaggtactttaaagccattaaaacatgttgatatggagccaatgactgatgcgttcttaactgcatgtgttgttgccgctatttcgcacgacagtgatccaaattctgcaaatacaaccaccattgaaggtattgcaaaccagcgtgtcaaagagtgtaacagaattttggccatggctacagagctcgccaaatttggcgtcaaaactacagaattaccagatggtattcaagtccatggtttaaactcgataaaagatttgaaggttccttccgactcttctggacctgtcggtgtatgcacatatgatgatcatcgtgtggccatgagtttctcgcttcttgcaggaatggtaaattctcaaaatgaacgtgacgaagttgctaatcctgtaagaatacttgaaagacattgtactggtaaaacctggcctggctggtgggatgtgttacattccgaactaggtgccaaattagatggtgcagaacctttagagtgcacatccaaaaagaactcaaagaaaagcgttgtcattattggcatgagagcagctggcaaaactactataagtaaatggtgcgcatccgctctgggttacaaattagttgacctagacgagctgtttgagcaacagcataacaatcaaagtgttaaacaatttgttgtggagaacggttgggagaagttccgtgaggaagaaacaagaattttcaaggaagttattcaaaattacggcgatgatggatatgttttctcaacaggtggcggtattgttgaaagcgctgagtctagaaaagccttaaaagattttgcctcatcaggtggatacgttttacacttacatagggatattgaggagacaattgtctttttacaaagtgatccttcaagacctgcctatgtggaagaaattcgtgaagtttggaacagaagggaggggtggtataaagaatgctcaaatttctctttctttgctcctcattgctccgcagaagctgagttccaagctctaagaagatcgtttagtaagtacattgcaaccattacaggtgtcagagaaatagaaattccaagcggaagatctgcctttgtgtgtttaacctttgatgacttaactgaacaaactgagaatttgactccaatctgttatggttgtgaggctgtagaggtcagagtagaccatttggctaattactctgctgatttcgtgagtaaacagttatctatattgcgtaaagccactgacagtattcctatcatttttactgtgcgaaccatgaagcaaggtggcaactttcctgatgaagagttcaaaaccttgagagagctatacgatattgccttgaagaatggtgttgaattccttgacttagaactaactttacctactgatatccaatatgaggttattaacaaaaggggcaacaccaagatcattggttcccatcatgacttccaaggattatactcctgggacgacgctgaatgggaaaacagattcaatcaagcgttaactcttgatgtggatgttgtaaaatttgtgggtacggctgttaatttcgaagataatttgagactggaacactttagggatacacacaagaataagcctttaattgcagttaatatgacttctaaaggtagcatttctcgtgttttgaataatgttttaacacctgtgacatcagatttattgcctaactccgctgcccctggccaattgacagtagcacaaattaacaagatgtatacatctatgggaggtatcgagcctaaggaactgtttgttgttggaaagccaattggccactctagatcgccaattttacataacactggctatgaaattttaggtttacctcacaagttcgataaatttgaaactgaatccgcacaattggtgaaagaaaaacttttggacggaaacaagaactttggcggtgctgcagtcacaattcctctgaaattagatataatgcagtacatggatgaattgactgatgctgctaaagttattggtgctgtaaacacagttataccattgggtaacaagaagtttaagggtgataataccgactggttaggtatccgtaatgccttaattaacaatggcgttcccgaatatgttggtcataccgctggtttggttatcggtgcaggtggcacttctagagccccactttacgccttgcacagtttaggttgcaaaaagatcttcataatcaacaggacaacttcgaaattgaagccattaatagagtcacttccatctgaattcaacattattggaatagagtccactaaatctatagaagagattaaggaacacgttggcgttgctgtcagctgtgtaccagccgacaaaccattagatgacgaacttttaagtaagctggagagattccttgtgaaaggtgcccatgctgcttttgtaccaaccttattggaagccgcatacaaaccaagcgttactcccgttatgacaatttcacaagacaaatatcaatggcacgttgtccctggatcacaaatgttagtacaccaaggtgtagctcagtttgaaaagtggacaggattcaagggccctttcaaggccatttttgatgccgttacgaaagagtag

SEQ ID NO: 24 - protein, 1588 aa, Artificial sequence
  Synthetic polypeptide
MVQLAKVPILGNDIIHVGYNIHDHLVETIIKHCPSSTYVICNDTNLSKVPYYQQLVLEFKASLPEGSRLLTYVVKPGETSKSRETKAQLEDYLLVEGCTRDTVMVAIGGGVIGDMIGFVASTFMRGVRVVQVPTSLLAMVDSSIGGKTAIDTPLGKNFIGAFWQPKFVLVDIKWLETLAKREFINGMAEVIKTACIWNADEFTRLESNASLFLNVVNGAKNVKVTNQLTNEIDEISNTDIEAMLDHTYKLVLESIKVKAEVVSSDERESSLRNLLNFGHSIGHAYEAILTPQALHGECVSIGMVKEAELSRYFGILSPTQVARLSKILVAYGLPVSPDEKWFKELTLHKKTPLDILLKKMSIDKKNEGSKKKVVILESIGKCYGDSAQFVSDEDLRFILTDETLVYPFKDIPADQQKVVIPPGSKSISNRALILAALGEGQCKIKNLLHSDDTKHMLTAVHELKGATISWEDNGETVVVEGHGGSTLSACADPLYLGNAGTASRFLTSLAALVNSTSSQKYIVLTGNARMQQRPIAPLVDSLRANGTKIEYLNNEGSLPIKVYTDSVFKGGRIELAATVSSQYVSSILMCAPYAEEPVTLALVGGKPISKLYVDMTIKMMEKFGINVETSTTEPYTYYIPKGHYINPSEYVIESDASSATYPLAFAAMTGTTVTVPNIGFESLQGDARFARDVLKPMGCKITQTATSTTVSGPPVGTLKPLKHVDMEPMTDAFLTACVVAAISHDSDPNSANTTTIEGIANQRVKECNRILAMATELAKFGVKTTELPDGIQVHGLNSIKDLKVPSDSSGPVGVCTYDDHRVAMSFSLLAGMVNSQNERDEVANPVRILERHCTGKTWPGWWDVLHSELGAKLDGAEPLECTSKKNSKKSVVIIGMRAAGKTTISKWCASALGYKLVDLDELFEQQHNNQSVKQFVVENGWEKFREEETRIFKEVIQNYGDDGYVFSTGGGIVESAESRKALKDFASSGGYVLHLHRDIEETIVFLQSDPSRPAYVEEIREVWNRREGWYKECSNFSFFAPHCSAEAEFQALRRSFSKYIATITGVREIEIPSGRSAFVCLTFDDLTEQTENLTPICYGCEAVEVRVDHLANYSADFVSKQLSILRKATDSIPIIFTVRTMKQGGNFPDEEFKTLRELYDIALKNGVEFLDLELTLPTDIQYEVINKRGNTKIIGSHHDFQGLYSWDDAEWENRFNQALTLDVDVVKFVGTAVNFEDNLRLEHFRDTHKNKPLIAVNMTSKGSISRVLNNVLTPVTSDLLPNSAAPGQLTVAQINKMYTSMGGIEPKELFVVGKPIGHSRSPILHNTGYEILGLPHKFDKFETESAQLVKEKLLDGNKNFGGAAVTIPLKLDIMQYMDELTDAAKVIGAVNTVIPLGNKKFKGDNTDWLGIRNALINNGVPEYVGHTAGLVIGAGGTSRAPLYALHSLGCKKIFIINRTTSKLKPLIESLPSEFNIIGIESTKSIEEIKEHVGVAVSCVPADKPLDDELLSKLERFLVKGAHAAFVPTLLEAAYKPSVTPVMTISQDKYQWHVVPGSQMLVHQGVAQFEKWTGFKGPFKAIFDAVTKE

SEQ ID NO: 25 - DNA, 5064 bp, Artificial sequence
  Synthetic nucleic acid
atggtgcagttagccaaagtcccaattctaggaaatgatattatccacgttgggtataacattcatgaccatttggttgaaaccataattaaacattgtccttcttcgacatacgttatttgcaatgatacgaacttgagtaaagttccatactaccagcaattagtcctggaattcaaggcttctttgccagaaggctctcgtttacttacttatgttgttaaaccaggtgagacaagtaaaagtagagaaaccaaagcgcagctagaagattatcttttagtggaaggatgtactcgtgatacggttatggtagcgatcggtggtggtgttattggtgacatgattgggttcgttgcatctacatttatgagaggtgttcgtgttgtccaagtaccaacatccttattggcaatggtcgattcctccattggtggtaaaactgctattgacactcctctaggtaaaaactttattggtgcattttggcaaccaaaatttgtccttgtagatattaaatggctagaaacgttagccaagagagagtttatcaatgggatggcagaagttatcaagactgcttgtatttggaacgctgacgaatttactagattagaatcaaacgcttcgttgttcttaaatgttgttaatggggcaaaaaatgtcaaggttaccaatcaattgacaaacgagattgacgagatatcgaatacagatattgaagctatgttggatcatacatataagttagttcttgagagtattaaggtcaaagcggaagttgtctcttcggatgaacgtgaatccagtctaagaaaccttttgaacttcggacattctattggtcatgcttatgaagctatactaaccccacaagcattacatggtgaatgtgtgtccattggtatggttaaagaggcggaattatcccgttatttcggtattctctcccctacccaagttgcacgtctatccaagattttggttgcctacgggttgcctgtttcgcctgatgagaaatggtttaaagagctaaccttacataagaaaacaccattggatatcttattgaagaaaatgagtattgacaagaaaaacgagggttccaaaaagaaggtggtcattttagaaagtattggtaagtgctatggtgactccgctcaatttgttagcgatgaagacctgagatttattctaacagatgaaaccctcgtttaccccttcaaggacatccctgctgatcaacagaaagttgttatcccccctggttctaagtccatctccaatcgtgctttaattcttgctgccctcggtgaaggtcaatgtaaaatcaagaacttattacattctgatgatactaaacatatgttaaccgctgttcatgaattgaaaggtgctacgatatcatgggaagataatggtgagacggtagtggtggaaggacatggtggttccacattgtcagcttgtgctgaccccttatatctaggtaatgcaggtactgcatctagatttttgacttccttggctgccttggtcaattctacttcaagccaaaagtatatcgttttaactggtaacgcaagaatgcaacaaagaccaattgctcctttggtcgattctttgcgtgctaatggtactaaaattgagtacttgaataatgaaggttccctgccaatcaaagtttatactgattcggtattcaaaggtggtagaattgaattagctgctacagtttcttctcagtacgtatcctctatcttgatgtgtgccccatacgctgaagaacctgtaactttggctcttgttggtggtaagccaatctctaaattgtacgtcgatatgacaataaaaatgatggaaaaattcggtatcaatgttgaaacttctactacagaaccttacacttattatattccaaagggacattatattaacccatcagaatacgtcattgaaagtgatgcctcaagtgctacatacccattggccttcgccgcaatgactggtactaccgtaacggttccaaacattggttttgagtcgttacaaggtgatgccagatttgcaagagatgtcttgaaacctatgggttgtaaaataactcaaacggcaacttcaactactgtttcgggtcctcctgtaggtactttaaagccattaaaacatgttgatatggagccaatgactgatgcgttcttaactgcatgtgttgttgccgctatttcgcacgacagtgatccaaattctgcaaatacaaccaccattgaaggtattgcaaaccagcgtgtcaaagagtgtaacagaattttggccatggctacagagctcgccaaatttggcgtcaaaactacagaattaccagatggtattcaagtccatggtttaaactcgataaaagatttgaaggttccttccgactcttctggacctgtcggtgtatgcacatatgatgatcatcgtgtggccatgagtttctcgcttcttgcaggaatggtaaattctcaaaatgaacgtgacgaagttgctaatcctgtaagaatacttgaaagacattgtactggtaaaacctggcctggctggtgggatgtgttacattccgaactaggtgccaaattagatggtgcagaacctttagagtgcacatccaaaaagaactcaaagaaaagcgttgtcattattggcatgagagcagctggcaaaactactataagtaaatggtgcgcatccgctctgggttacaaattagttgacctagacgagctgtttgagcaacagcataacaatcaaagtgttaaacaatttgttgtggagaacggttgggagaagttccgtgaggaagaaacaagaattttcaaggaagttattcaaaattacggcgatgatggatatgttttctcaacaggtggcggtattgttgaaagcgctgagtctagaaaagccttaaaagattttgcctcatcaggtggatacgttttacacttacatagggatattgaggagacaattgtctttttacaaagtgatccttcaagacctgcctatgtggaagaaattcgtgaagtttggaacagaagggaggggtggtataaagaatgctcaaatttctctttctttgctcctcattgctccgcagaagctgagttccaagctctaagaagatcgtttagtaagtacattgcaaccattacaggtgtcagagaaatagaaattccaagcggaagatctgcctttgtgtgtttaacctttgatgacttaactgaacaaactgagaatttgactccaatctgttatggttgtgaggctgtagaggtcagagtagaccatttggctaattactctgctgatttcgtgagtaaacagttatctatattgcgtaaagccactgacagtattcctatcatttttactgtgcgaaccatgaagcaaggtggcaactttcctgatgaagagttcaaaaccttgagagagctatacgatattgccttgaagaatggtgttgaattccttgacttagaactaactttacctactgatatccaatatgaggttattaacaaaaggggcaacaccaagatcattggttcccatcatgacttccaaggattatactcctgggacgacgctgaatgggaaaacagattcaatcaagcgttaactcttgatgtggatgttgtaaaatttgtgggtacggctgttaatttcgaagataatttgagactggaacactttagggatacacacaagaataagcctttaattgcagttaatatgacttctaaaggtagcatttctcgtgttttgaataatgttttaacacctgtgacatcagatttattgcctaactccgctgcccctggccaattgacagtagcacaaattaacaagatgtatacatctatgggaggtatcgagcctaaggaactgtttgttgttggaaagccaattggccccgggaaaatgccttccaaactcgccatcacttccatgtcacttggccggtgttatgccggccactccttcaccactaagctcgatatggcccggaaatatggctatcaaggcctagagctcttccacgaggacttggctgatgtagcctatcgtctctccggagagaccccttccccatgtggcccgtccccagcagcccagctctcggctgcccgtcaaatcctccgcatgtgccaagtcagaaacattgaaatcgtctgcctccagcccttcagccagtacgacggcctactcgaccgcgaggagcacgagcgccgtctggagcagctcgagttctggatcgagctcgcccacgagcttgacacagacattatccaaatccccgccaactttctccccgccgaggaagtaactgaggacatttcgctcatcgtctcggaccttcaagaagtggccgacatgggcctgcaggccaacccacccatccgctttgtctacgaggctctgtgctggagcactcgtgtcgacacttgggagcgtagctgggaggtggtgcagagggtgaacaggcccaactttggcgtgtgcctggacactttcaacattgcggggcgggtatatgctgatccgacggttgcctctggccgcacccccaacgcggaggaagcgatacggaagtcgattgcgcgtctcgttgaaagggtcgatgtcagcaaggtcttttatgtgcaggttgtggacgctgagaagttgaagaagccgctggtgccgggtcatcggttttatgacccggagcagccggcgaggatgagctggtcaaggaactgcaggttattctacggggagaaggacagaggggcgtatttgcccgtcaaggagattgcctgggccttcttcaacgggctcggattcgagggttgggtcagtctggagctcttcaacagaagaatgtcggacacaggctttggggtgcccgaggagctggccaggagaggggccgtgtcgtgggcaaagctggtgagggacatgaagatcactgttgattcaccaacacaacaacaagccacacagcagcccatcaggatgctgtcgctgtcagcggctttgtaa

SEQ ID NO: 26 - protein, 1687 aa, Artificial sequence
  Synthetic polypeptide
MVQLAKVPILGNDIIHVGYNIHDHLVETIIKHCPSSTYVICNDTNLSKVPYYQQLVLEFKASLPEGSRLLTYVVKPGETSKSRETKAQLEDYLLVEGCTRDTVMVAIGGGVIGDMIGFVASTFMRGVRVVQVPTSLLAMVDSSIGGKTAIDTPLGKNFIGAFWQPKFVLVDIKWLETLAKREFINGMAEVIKTACIWNADEFTRLESNASLFLNVVNGAKNVKVTNQLTNEIDEISNTDIEAMLDHTYKLVLESIKVKAEVVSSDERESSLRNLLNFGHSIGHAYEAILTPQALHGECVSIGMVKEAELSRYFGILSPTQVARLSKILVAYGLPVSPDEKWFKELTLHKKTPLDILLKKMSIDKKNEGSKKKVVILESIGKCYGDSAQFVSDEDLRFILTDETLVYPFKDIPADQQKVVIPPGSKSISNRALILAALGEGQCKIKNLLHSDDTKHMLTAVHELKGATISWEDNGETVVVEGHGGSTLSACADPLYLGNAGTASRFLTSLAALVNSTSSQKYIVLTGNARMQQRPIAPLVDSLRANGTKIEYLNNEGSLPIKVYTDSVFKGGRIELAATVSSQYVSSILMCAPYAEEPVTLALVGGKPISKLYVDMTIKMMEKFGINVETSTTEPYTYYIPKGHYINPSEYVIESDASSATYPLAFAAMTGTTVTVPNIGFESLQGDARFARDVLKPMGCKITQTATSTTVSGPPVGTLKPLKHVDMEPMTDAFLTACVVAAISHDSDPNSANTTTIEGIANQRVKECNRILAMATELAKFGVKTTELPDGIQVHGLNSIKDLKVPSDSSGPVGVCTYDDHRVAMSFSLLAGMVNSQNERDEVANPVRILERHCTGKTWPGWWDVLHSELGAKLDGAEPLECTSKKNSKKSVVIIGMRAAGKTTISKWCASALGYKLVDLDELFEQQHNNQSVKQFVVENGWEKFREEETRIFKEVIQNYGDDGYVFSTGGGIVESAESRKALKDFASSGGYVLHLHRDIEETIVFLQSDPSRPAYVEEIREVWNRREGWYKECSNFSFFAPHCSAEAEFQALRRSFSKYIATITGVREIEIPSGRSAFVCLTFDDLTEQTENLTPICYGCEAVEVRVDHLANYSADFVSKQLSILRKATDSIPIIFTVRTMKQGGNFPDEEFKTLRELYDIALKNGVEFLDLELTLPTDIQYEVINKRGNTKIIGSHHDFQGLYSWDDAEWENRFNQALTLDVDVVKFVGTAVNFEDNLRLEHFRDTHKNKPLIAVNMTSKGSISRVLNNVLTPVTSDLLPNSAAPGQLTVAQINKMYTSMGGIEPKELFVVGKPIGPGKMPSKLAITSMSLGRCYAGHSFTTKLDMARKYGYQGLELFHEDLADVAYRLSGETPSPCGPSPAAQLSAARQILRMCQVRNIEIVCLQPFSQYDGLLDREEHERRLEQLEFWIELAHELDTDIIQIPANFLPAEEVTEDISLIVSDLQEVADMGLQANPPIRFVYEALCWSTRVDTWERSWEVVQRVNRPNFGVCLDTFNIAGRVYADPTVASGRTPNAEEAIRKSIARLVERVDVSKVFYVQVVDAEKLKKPLVPGHRFYDPEQPARMSWSRNCRLFYGEKDRGAYLPVKEIAWAFFNGLGFEGWVSLELFNRRMSDTGFGVPEELARRGAVSWAKLVRDMKITVDSPTQQQATQQPIRMLSLSAAL

SEQ ID NO: 27 - protein, 221 aa, Homo sapiens
MGDTKEQRILNHVLQHAEPGNAQSVLEAIDTYCEQKEWAMNVGDKKGKIVDAVIQEHQPSVLLELGAYCGYSAVRMARLLSPGARLITIEINPDCAAITQRMVDFAGVKDKVTLVVGASQDIIPQLKKKYDVDTLDMVFLDHWKDRYLPDTLLLEECGLLRKGTVLLADNVICPGAPDFLAHVRGSSCFECTHYQSFLEYREVVDGLEKAIYKGPGSEAGP

SEQ ID NO: 28 - DNA, 40 bp, Artificial sequence
  Synthetic oligonucleotide
cgtagcatgcagtctagaaaaatgggtgacactaaggagc

SEQ ID NO: 29 - DNA, 45 bp, Artificial sequence
  Synthetic oligonucleotide
gacgacgttagtgacagaattcttatggaccagcttcagaacctg

SEQ ID NO: 30 - DNA, 25 bp, Artificial sequence
  Synthetic oligonucleotide
cgtagcatgcagtctagaaaaatgg

SEQ ID NO: 31 - DNA, 22 bp, Artificial sequence
  Synthetic oligonucleotide
gacgacgttagtgacagaattc

SEQ ID NO: 32 - DNA, 45 bp, Artificial sequence
  Synthetic oligonucleotide
  misc_feature (30)..(30): n is a, c, g, or t
ctattgacacttattgtgagcaaaaggagnrkgctatgaacgttg

SEQ ID NO: 33 - DNA, 45 bp, Artificial sequence
  Synthetic oligonucleotide
  misc_feature (30)..(30): n is a, c, g, or t
ctattgacacttattgtgagcaaaaggagnykgctatgaacgttg

SEQ ID NO: 34 - DNA, 29 bp, Artificial sequence
  Synthetic oligonucleotide
ctccttttgctcacaataagtgtcaatag

SEQ ID NO: 35 - DNA, 45 bp, Artificial sequence
  Synthetic oligonucleotide
  misc_feature (31)..(31): n is a, c, g, or t
gacacttattgtgagcaaaaggagtgggctnrkaacgttggtgac

SEQ ID NO: 36 - DNA, 43 bp, Artificial sequence
  Synthetic oligonucleotide
  misc_feature (29)..(29): n is a, c, g, or t
cacttattgtgagcaaaaggagtgggctnykaacgttggtgac

SEQ ID NO: 37 - DNA, 24 bp, Artificial sequence
  Synthetic oligonucleotide
ctccttttgctcacaataagtgtc

SEQ ID NO: 38 - DNA, 46 bp, Artificial sequence
  Synthetic oligonucleotide
  misc_feature (27)..(27): n is a, c, g, or t
ctttggacatggttttcttggaccatnrkaaggacagatatttgcc

SEQ ID NO: 39 - DNA, 46 bp, Artificial sequence
  Synthetic oligonucleotide
  misc_feature (27)..(27): n is a, c, g, or t
ctttggacatggttttcttggaccatnykaaggacagatatttgcc

SEQ ID NO: 40 - DNA, 26 bp, Artificial sequence
  Synthetic oligonucleotide
atggtccaagaaaaccatgtccaaag

SEQ ID NO: 41 - DNA, 53 bp, Artificial sequence
  Synthetic oligonucleotide
  misc_feature (30)..(30): n is a, c, g, or t
gtactgttttgttagctgacaacgttattnrkccaggtgctccagacttcttg

SEQ ID NO: 42 - DNA, 53 bp, Artificial sequence
  Synthetic oligonucleotide
  misc_feature (30)..(30): n is a, c, g, or t
gtactgttttgttagctgacaacgttattnykccaggtgctccagacttcttg

SEQ ID NO: 43 - DNA, 29 bp, Artificial sequence
  Synthetic oligonucleotide
aataacgttgtcagctaacaaaacagtac

SEQ ID NO: 44 - DNA, 47 bp, Artificial sequence
  Synthetic oligonucleotide
  misc_feature (30)..(30): n is a, c, g, or t
ctgttttgttagctgacaacgttatttgtnrkggtgctccagacttc

SEQ ID NO: 45 - DNA, 47 bp, Artificial sequence
  Synthetic oligonucleotide
  misc_feature (30)..(30): n is a, c, g, or t
ctgttttgttagctgacaacgttatttgtnykggtgctccagacttc

SEQ ID NO: 46 - DNA, 29 bp, Artificial sequence
  Synthetic oligonucleotide
acaaataacgttgtcagctaacaaaacag

SEQ ID NO: 47 - DNA, 103 bp, Artificial sequence
  Synthetic oligonucleotide
  misc_feature (86)..(86): n is a, c, g, or t
atttagaattcttatggaccagcttcagaacctggacccttatatatagccttctccaaaccgtcaacaacctctctatattcmyngaaagattgataatgag

SEQ ID NO: 48 - DNA, 102 bp, Artificial sequence
  Synthetic oligonucleotide
  misc_feature (85)..(85): n is a, c, g, or t
atttagaattctatggaccagcttcagaacctggacccttatatatagccttctccaaaccgtcaacaacctctctatattcmrngaaagattgataatgag

SEQ ID NO: 49 - DNA, 101 bp, Artificial sequence
  Synthetic oligonucleotide
  misc_feature (83)..(83): n is a, c, g, or t
atttagaattcttatggaccagcttcagaacctggacccttatatatagccttctccaaaccgtcaacaacctctctatamyncaagaaagattgataatg

SEQ ID NO: 50 - DNA, 101 bp, Artificial sequence
  Synthetic oligonucleotide
  misc_feature (83)..(83): n is a, c, g, or t
atttagaattcttatggaccagcttcagaacctggacccttatatatagccttctccaaaccgtcaacaacctctctatamrncaagaaagattgataatg

SEQ ID NO: 51 - DNA, 95 bp, Artificial sequence
  Synthetic oligonucleotide
  misc_feature (77)..(77): n is a, c, g, or t
atttagaattcttatggaccagcttcagaacctggacccttatatatagccttctccaaaccgtcaacaacctcmynatattccaagaaagattg

SEQ ID NO: 52 - DNA, 95 bp, Artificial sequence
  Synthetic oligonucleotide
  misc_feature (77)..(77): n is a, c, g, or t
atttagaattcttatggaccagcttcagaacctggacccttatatatagccttctccaaaccgtcaacaacctcmrnatattccaagaaagattg

SEQ ID NO: 53 - protein, 363 aa, Arabidopsis thaliana
MGSTAETQLTPVQVTDDEAALFAMQLASASVLPMALKSALELDLLEIMAKNGSPMSPTEIASKLPTKNPEAPVMLDRILRLLTSYSVLTCSNRKLSGDGVERIYGLGPVCKYLTKNEDGVSIAALCLMNQDKVLMESWYHLKDAILDGGIPFNKAYGMSAFEYHGTDPRFNKVFNNGMSNHSTITMKKILETYKGFEGLTSLVDVGGGIGATLKMIVSKYPNLKGINFDLPHVIEDAPSHPGIEHVGGDMFVSVPKGDAIFMKWICHDWSDEHCVKFLKNCYESLPEDGKVILAECILPETPDSSLSTKQVVHVDCIMLAHNPGGKERTEKEFEALAKASGFKGIKVVCDAFGVNLIELLKKL

SEQ ID NO: 54 - protein, 365 aa, Fragaria x ananassa
MGSTGETQMTPTHVSDEEANLFAMQLASASVLPMVLKAAIELDLLEIMAKAGPGSFLSPSDLASQLPTKNPEAPVMLDRMLRLLASYSILTCSLRTLPDGKVERLYCLGPVCKFLTKNEDGVSIAALCLMNQDKVLVESWYHLKDAVLDGGIPFNKAYGMTAFDYHGTDPRFNKVFNKGMADHSTITMKKILETYKGFEGLKSIVDVGGGTGAVVNMIVSKYPSIKGINFDLPHVIEDAPQYPGVQHVGGDMFVSVPKGNAIFMKWICHDWSDEHCIKFLKNCYAALPDDGKVILAECILPVAPDTSLATKGVVHMDVIMLAHNPGGKERTEQEFEALAKGSGFQGIRVCCDAFNTYVIEFLKKI

SEQ ID NO: 55 - protein, 271 aa, Homo sapiens
MPEAPPLLLAAVLLGLVLLVVLLLLLRHWGWGLCLIGWNEFILQPIHNLLMGDTKEQRILNHVLQHAEPGNAQSVLEAIDTYCEQKEWAMNVGDKKGKIVDAVIQEHQPSVLLELGAYCGYSAVRMARLLSPGARLITIEINPDCAAITQRMVDFAGVKDKVTLVVGASQDIIPQLKKKYDVDTLDMVFLDHWKDRYLPDTLLLEECGLLRKGTVLLADNVICPGAPDFLAHVRGSSCFECTHYQSFLEYREVVDGLEKAIYKGPGSEAGP

SEQ ID NO: 56 - protein, 263 aa, Vanilla planifolia
MATTVATATRATENKTQTEENSQNGGQQTGHQEIGHKSLLKSDALYQYILETSVYPREPECLKELREITAKHPWNLMTTSADEGQFLGMLLKLINAKNTMEIGVFTGYSLLATALALPDDGKILAMDINRENYELGLPLIQKAGVAHKIDFREGPALPVLDELMKDESKHGSFDFIFVDADKDNYLNYHQRIIDLVKVGGVIGYDNTLWNGAVVLPPDAPMRKYIRYYRDFVIELNKELAADPRIEICQLPVGDGITLCRRVK